European Patent Application EP 4 620 978 A1, published September 24, 2025. Title: UNIVERSAL CAR-T CELL TARGETING B7H3, AND PREPARATION METHOD THEREFOR AND USE THEREOF. Applicant: T-MAXIMUM Pharmaceutical (Suzhou) Co., Ltd. The sequence listing filed with the application follows.

SEQUENCE LISTING (244 sequences)

SEQ ID NO: 1 - protein, 8 aa, synthetic construct
  REGION 1..8: note = 1G7 HCDR1hu1G7 HCDR1
GRIFSNYA

SEQ ID NO: 2 - protein, 8 aa, synthetic construct
  REGION 1..8: note = 1A5 HCDR1hu1A5 HCDR1
GRIFSNYS

SEQ ID NO: 3 - protein, 8 aa, synthetic construct
  REGION 1..8: note = 1G7 HCDR2hu1G7 HCDR2
IIGSTGTV

SEQ ID NO: 4 - protein, 8 aa, synthetic construct
  REGION 1..8: note = 1A5 HCDR2hu1A5 HCDR2
IIWSTGTT

SEQ ID NO: 5 - protein, 18 aa, synthetic construct
  REGION 1..18: note = 1G7 HCDR3hu1G7 HCDR3
AASFRYSGIYGREADFVS

SEQ ID NO: 6 - protein, 18 aa, synthetic construct
  REGION 1..18: note = 1A5 HCDR3hu1A5 HCDR3
AASFKYSGIYGREADFGS

SEQ ID NO: 7 - protein, 25 aa, synthetic construct
  REGION 1..25: note = 1G7 HFR1
AVQLVESGGGLVQTGGSLRLSCADS

SEQ ID NO: 8 - protein, 25 aa, synthetic construct
  REGION 1..25: note = hu1G7 HFR1
AVQLVESGGGLVQPGGSLRLSCAAS

SEQ ID NO: 9 - protein, 25 aa, synthetic construct
  REGION 1..25: note = 1A5 HFR1
QAQLVESGGGLVQTGGSLRLSCAAS

SEQ ID NO: 10 - protein, 25 aa, synthetic construct
  REGION 1..25: note = hu1A5 HFR1
QVQLVESGGGLVQPGGSLRLSCAAS

SEQ ID NO: 11 - protein, 17 aa, synthetic construct
  REGION 1..17: note = 1G7 HFR2hu1G7 HFR2
MGWFRQAPGKEREFVAA

SEQ ID NO: 12 - protein, 17 aa, synthetic construct
  REGION 1..17: note = 1A5 HFR2hu1A5 HFR2
VGWFRQAPGKEREFVAA

SEQ ID NO: 13 - protein, 38 aa, synthetic construct
  REGION 1..38: note = 1G7 HFR3
NYADSMKGRFTISRDNAKNTVVLQMNSLKPEDTAIYYC

SEQ ID NO: 14 - protein, 38 aa, synthetic construct
  REGION 1..38: note = hu1G7 HFR3hu1A5 HFR3
YYADSVKGRFTISRDNSKNTLYLQMNSLRAEDTAVYYC

SEQ ID NO: 15 - protein, 38 aa, synthetic construct
  REGION 1..38: note = 1A5 HFR3
NLADPMKGRFTISRDNAKNTVVLQMNSLKPEDTAIYYC

SEQ ID NO: 16 - protein, 11 aa, synthetic construct
  REGION 1..11: note = 1G7 HFR41A5 HFR4
WGQGTQVTVSS

SEQ ID NO: 17 - protein, 11 aa, synthetic construct
  REGION 1..11: note = hu1G7 HFR4hu1A5 HFR4
WGQGTLVTVSS

SEQ ID NO: 18 - protein, 125 aa, synthetic construct
  REGION 1..125: note = 1G7 VHH
AVQLVESGGGLVQTGGSLRLSCADSGRIFSNYAMGWFRQAPGKEREFVAAIIGSTGTVNYADSMKGRFTISRDNAKNTVVLQMNSLKPEDTAIYYCAASFRYSGIYGREADFVSWGQGTQVTVSS

SEQ ID NO: 19 - protein, 125 aa, synthetic construct
  REGION 1..125: note = hu1G7 VHH
AVQLVESGGGLVQPGGSLRLSCAASGRIFSNYAMGWFRQAPGKEREFVAAIIGSTGTVYYADSVKGRFTISRDNSKNTLYLQMNSLRAEDTAVYYCAASFRYSGIYGREADFVSWGQGTLVTVSS

SEQ ID NO: 20 - protein, 125 aa, synthetic construct
  REGION 1..125: note = 1A5 VHH
QAQLVESGGGLVQTGGSLRLSCAASGRIFSNYSVGWFRQAPGKEREFVAAIIWSTGTTNLADPMKGRFTISRDNAKNTVVLQMNSLKPEDTAIYYCAASFKYSGIYGREADFGSWGQGTQVTVSS

SEQ ID NO: 21 - protein, 125 aa, synthetic construct
  REGION 1..125: note = hu1A5 VHH
QVQLVESGGGLVQPGGSLRLSCAASGRIFSNYSVGWFRQAPGKEREFVAAIIWSTGTTYYADSVKGRFTISRDNSKNTLYLQMNSLRAEDTAVYYCAASFKYSGIYGREADFGSWGQGTLVTVSS

SEQ ID NO: 22 - protein, 15 aa, synthetic construct
  REGION 1..15: note = Linker
GGGGSGGGGSGGGGS

SEQ ID NO: 23 - protein, 265 aa, synthetic construct
  REGION 1..265: note = 1G7-1A5
AVQLVESGGGLVQTGGSLRLSCADSGRIFSNYAMGWFRQAPGKEREFVAAIIGSTGTVNYADSMKGRFTISRDNAKNTVVLQMNSLKPEDTAIYYCAASFRYSGIYGREADFVSWGQGTQVTVSSGGGGSGGGGSGGGGSQAQLVESGGGLVQTGGSLRLSCAASGRIFSNYSVGWFRQAPGKEREFVAAIIWSTGTTNLADPMKGRFTISRDNAKNTVVLQMNSLKPEDTAIYYCAASFKYSGIYGREADFGSWGQGTQVTVSS

SEQ ID NO: 24 - protein, 265 aa, synthetic construct
  REGION 1..265: note = Hu1G7-Hu1A5
AVQLVESGGGLVQPGGSLRLSCAASGRIFSNYAMGWFRQAPGKEREFVAAIIGSTGTVYYADSVKGRFTISRDNSKNTLYLQMNSLRAEDTAVYYCAASFRYSGIYGREADFVSWGQGTLVTVSSGGGGSGGGGSGGGGSQVQLVESGGGLVQPGGSLRLSCAASGRIFSNYSVGWFRQAPGKEREFVAAIIWSTGTTYYADSVKGRFTISRDNSKNTLYLQMNSLRAEDTAVYYCAASFKYSGIYGREADFGSWGQGTLVTVSS

SEQ ID NO: 25 - protein, 265 aa, synthetic construct
  REGION 1..265: note = 1A5-1G7
QAQLVESGGGLVQTGGSLRLSCAASGRIFSNYSVGWFRQAPGKEREFVAAIIWSTGTTNLADPMKGRFTISRDNAKNTVVLQMNSLKPEDTAIYYCAASFKYSGIYGREADFGSWGQGTQVTVSSGGGGSGGGGSGGGGSAVQLVESGGGLVQTGGSLRLSCADSGRIFSNYAMGWFRQAPGKEREFVAAIIGSTGTVNYADSMKGRFTISRDNAKNTVVLQMNSLKPEDTAIYYCAASFRYSGIYGREADFVSWGQGTQVTVSS

SEQ ID NO: 26 - protein, 265 aa, synthetic construct
  REGION 1..265: note = Hu1A5-Hu1G7
QVQLVESGGGLVQPGGSLRLSCAASGRIFSNYSVGWFRQAPGKEREFVAAIIWSTGTTYYADSVKGRFTISRDNSKNTLYLQMNSLRAEDTAVYYCAASFKYSGIYGREADFGSWGQGTLVTVSSGGGGSGGGGSGGGGSAVQLVESGGGLVQPGGSLRLSCAASGRIFSNYAMGWFRQAPGKEREFVAAIIGSTGTVYYADSVKGRFTISRDNSKNTLYLQMNSLRAEDTAVYYCAASFRYSGIYGREADFVSWGQGTLVTVSS

SEQ ID NO: 27 - protein, 237 aa, synthetic construct
  REGION 1..237: note = The amino acid sequence of the non-antigen binding domain of CAR
FVPVFLPAKPTTTPAPRPPTPAPTIASQPLSLRPEACRPAAGGAVHTRGLDFACDIYIWAPLAGTCGVLLLSLVITLYCNHRNKRGRKKLLYIFKQPFMRPVQTTQEEDGCSCRFPEEEEGGCELRVKFSRSADAPAYQQGQNQLYNELNLGRREEYDVLDKRRGRDPEMGGKPRRKNPQEGLYNELQKDKMAEAYSEIGMKGERRRGKGHDGLYQGLSTATKDTYDALHMQALPPR

SEQ ID NO: 28 - protein, 21 aa, synthetic construct
  REGION 1..21: note = The amino acid sequence of CD8A signal peptide
MALPVTALLLPLALLLHAARP

SEQ ID NO: 29 - protein, 383 aa, synthetic construct
  REGION 1..383: note = The amino acid sequence of 1G7 CAR
MALPVTALLLPLALLLHAARPAVQLVESGGGLVQTGGSLRLSCADSGRIFSNYAMGWFRQAPGKEREFVAAIIGSTGTVNYADSMKGRFTISRDNAKNTVVLQMNSLKPEDTAIYYCAASFRYSGIYGREADFVSWGQGTQVTVSSFVPVFLPAKPTTTPAPRPPTPAPTIASQPLSLRPEACRPAAGGAVHTRGLDFACDIYIWAPLAGTCGVLLLSLVITLYCNHRNKRGRKKLLYIFKQPFMRPVQTTQEEDGCSCRFPEEEEGGCELRVKFSRSADAPAYQQGQNQLYNELNLGRREEYDVLDKRRGRDPEMGGKPRRKNPQEGLYNELQKDKMAEAYSEIGMKGERRRGKGHDGLYQGLSTATKDTYDALHMQALPPR

SEQ ID NO: 30 - protein, 383 aa, synthetic construct
  REGION 1..383: note = The amino acid sequence of Hu1G7 CAR
MALPVTALLLPLALLLHAARPAVQLVESGGGLVQPGGSLRLSCAASGRIFSNYAMGWFRQAPGKEREFVAAIIGSTGTVYYADSVKGRFTISRDNSKNTLYLQMNSLRAEDTAVYYCAASFRYSGIYGREADFVSWGQGTLVTVSSFVPVFLPAKPTTTPAPRPPTPAPTIASQPLSLRPEACRPAAGGAVHTRGLDFACDIYIWAPLAGTCGVLLLSLVITLYCNHRNKRGRKKLLYIFKQPFMRPVQTTQEEDGCSCRFPEEEEGGCELRVKFSRSADAPAYQQGQNQLYNELNLGRREEYDVLDKRRGRDPEMGGKPRRKNPQEGLYNELQKDKMAEAYSEIGMKGERRRGKGHDGLYQGLSTATKDTYDALHMQALPPR

SEQ ID NO: 31 - protein, 383 aa, synthetic construct
  REGION 1..383: note = The amino acid sequence of 1A5 CAR
MALPVTALLLPLALLLHAARPQAQLVESGGGLVQTGGSLRLSCAASGRIFSNYSVGWFRQAPGKEREFVAAIIWSTGTTNLADPMKGRFTISRDNAKNTVVLQMNSLKPEDTAIYYCAASFKYSGIYGREADFGSWGQGTQVTVSSFVPVFLPAKPTTTPAPRPPTPAPTIASQPLSLRPEACRPAAGGAVHTRGLDFACDIYIWAPLAGTCGVLLLSLVITLYCNHRNKRGRKKLLYIFKQPFMRPVQTTQEEDGCSCRFPEEEEGGCELRVKFSRSADAPAYQQGQNQLYNELNLGRREEYDVLDKRRGRDPEMGGKPRRKNPQEGLYNELQKDKMAEAYSEIGMKGERRRGKGHDGLYQGLSTATKDTYDALHMQALPPR

SEQ ID NO: 32 - protein, 383 aa, synthetic construct
  REGION 1..383: note = The amino acid sequence of Hu1A5 CAR
MALPVTALLLPLALLLHAARPQVQLVESGGGLVQPGGSLRLSCAASGRIFSNYSVGWFRQAPGKEREFVAAIIWSTGTTYYADSVKGRFTISRDNSKNTLYLQMNSLRAEDTAVYYCAASFKYSGIYGREADFGSWGQGTLVTVSSFVPVFLPAKPTTTPAPRPPTPAPTIASQPLSLRPEACRPAAGGAVHTRGLDFACDIYIWAPLAGTCGVLLLSLVITLYCNHRNKRGRKKLLYIFKQPFMRPVQTTQEEDGCSCRFPEEEEGGCELRVKFSRSADAPAYQQGQNQLYNELNLGRREEYDVLDKRRGRDPEMGGKPRRKNPQEGLYNELQKDKMAEAYSEIGMKGERRRGKGHDGLYQGLSTATKDTYDALHMQALPPR

SEQ ID NO: 33 - protein, 286 aa, synthetic construct
  REGION 1..286: note = The amino acid sequence of 1G7-1A5 CAR
MALPVTALLLPLALLLHAARPAVQLVESGGGLVQTGGSLRLSCADSGRIFSNYAMGWFRQAPGKEREFVAAIIGSTGTVNYADSMKGRFTISRDNAKNTVVLQMNSLKPEDTAIYYCAASFRYSGIYGREADFVSWGQGTQVTVSSGGGGSGGGGSGGGGSQAQLVESGGGLVQTGGSLRLSCAASGRIFSNYSVGWFRQAPGKEREFVAAIIWSTGTTNLADPMKGRFTISRDNAKNTVVLQMNSLKPEDTAIYYCAASFKYSGIYGREADFGSWGQGTQVTVSS

SEQ ID NO: 34 - protein, 287 aa, synthetic construct
  REGION 1..287: note = The amino acid sequence of Hu1G7-Hu1A5 CAR
MALPVTALLLPLALLLHAARPAAVQLVESGGGLVQPGGSLRLSCAASGRIFSNYAMGWFRQAPGKEREFVAAIIGSTGTVYYADSVKGRFTISRDNSKNTLYLQMNSLRAEDTAVYYCAASFRYSGIYGREADFVSWGQGTLVTVSSGGGGSGGGGSGGGGSQVQLVESGGGLVQPGGSLRLSCAASGRIFSNYSVGWFRQAPGKEREFVAAIIWSTGTTYYADSVKGRFTISRDNSKNTLYLQMNSLRAEDTAVYYCAASFKYSGIYGREADFGSWGQGTLVTVSS

SEQ ID NO: 35 - protein, 524 aa, synthetic construct
  REGION 1..524: note = The amino acid sequence of 1A5-1G7 CAR
MALPVTALLLPLALLLHAARPAQAQLVESGGGLVQTGGSLRLSCAASGRIFSNYSVGWFRQAPGKEREFVAAIIWSTGTTNLADPMKGRFTISRDNAKNTVVLQMNSLKPEDTAIYYCAASFKYSGIYGREADFGSWGQGTQVTVSSGGGGSGGGGSGGGGSAVQLVESGGGLVQTGGSLRLSCADSGRIFSNYAMGWFRQAPGKEREFVAAIIGSTGTVNYADSMKGRFTISRDNAKNTVVLQMNSLKPEDTAIYYCAASFRYSGIYGREADFVSWGQGTQVTVSSFVPVFLPAKPTTTPAPRPPTPAPTIASQPLSLRPEACRPAAGGAVHTRGLDFACDIYIWAPLAGTCGVLLLSLVITLYCNHRNKRGRKKLLYIFKQPFMRPVQTTQEEDGCSCRFPEEEEGGCELRVKFSRSADAPAYQQGQNQLYNELNLGRREEYDVLDKRRGRDPEMGGKPRRKNPQEGLYNELQKDKMAEAYSEIGMKGERRRGKGHDGLYQGLSTATKDTYDALHMQALPPR

SEQ ID NO: 36 - protein, 524 aa, synthetic construct
  REGION 1..524: note = The amino acid sequence of Hu1A5-Hu1G7 CAR
MALPVTALLLPLALLLHAARPAQVQLVESGGGLVQPGGSLRLSCAASGRIFSNYSVGWFRQAPGKEREFVAAIIWSTGTTYYADSVKGRFTISRDNSKNTLYLQMNSLRAEDTAVYYCAASFKYSGIYGREADFGSWGQGTLVTVSSGGGGSGGGGSGGGGSAVQLVESGGGLVQPGGSLRLSCAASGRIFSNYAMGWFRQAPGKEREFVAAIIGSTGTVYYADSVKGRFTISRDNSKNTLYLQMNSLRAEDTAVYYCAASFRYSGIYGREADFVSWGQGTLVTVSSFVPVFLPAKPTTTPAPRPPTPAPTIASQPLSLRPEACRPAAGGAVHTRGLDFACDIYIWAPLAGTCGVLLLSLVITLYCNHRNKRGRKKLLYIFKQPFMRPVQTTQEEDGCSCRFPEEEEGGCELRVKFSRSADAPAYQQGQNQLYNELNLGRREEYDVLDKRRGRDPEMGGKPRRKNPQEGLYNELQKDKMAEAYSEIGMKGERRRGKGHDGLYQGLSTATKDTYDALHMQALPPR

SEQ ID NO: 37 - DNA, 375 bp, synthetic construct
  misc_feature 1..375: note = Nucleotide sequence of 1G7 VHH
  source 1..375: mol_type = other DNA
gctgtccagcttgtggagtctggggggggcctcgtccagacaggcggttctctccgcctctcctgtgctgattctggcagaatcttttcaaactacgcaatgggctggttcaggcaggcaccaggcaaggagcgggagttcgtggctgctatcattggatctactggcaccgttaactacgcagacagcatgaaaggcagatttaccatctcaagagataacgccaaaaatactgtagtcctccagatgaactctctgaagcctgaggataccgctatatattattgtgcggcgtcattcaggtacagcggcatctatggccgcgaagcggattttgttagttggggacaagggacccaagtgacagtgtcttca

SEQ ID NO: 38 - DNA, 375 bp, synthetic construct
  misc_feature 1..375: note = Nucleotide sequence of hu1G7 VHH
  source 1..375: mol_type = other DNA
gctgttcagctggtggagtctggtggcgggctcgttcagccgggcggcagcctcagactgagctgtgcagcctccggaaggatcttttcaaattacgcaatggggtggtttaggcaggcaccaggaaaggagcgagagtttgtggcagcaataatcggttctaccggcacagtgtattacgctgatagcgtgaaaggcaggttcaccatttcaagggataacagtaaaaacacactatacttacagatgaactccttacgagccgaagacacggcggtgtactactgtgccgcatcctttagatactctggaatttacggacgcgaggccgactttgtcagctggggtcaggggactcttgttaccgtatcctct

SEQ ID NO: 39 - DNA, 375 bp, synthetic construct
  misc_feature 1..375: note = Nucleotide sequence of 1A5 VHH
  source 1..375: mol_type = other DNA
caggctcaactggtggagtcgggaggtggcttggtgcagacaggagggagcctgcgactctcctgtgcggcttccggaaggattttctctaattattctgtcggatggttccggcaggccccaggcaaagagcgtgaattcgttgcggcgataatctggtcgaccggaacaacgaatctggccgatcccatgaaggggagattcaccattagtagagacaacgcaaaaaacacagtagtcctgcagatgaacagcctcaaacccgaggatacagctatctattactgcgcagcttcctttaaatattctggcatatatggcagagaagcagattttgggagttgggggcagggcacccaggtgacagtcagttct

SEQ ID NO: 40 - DNA, 375 bp, synthetic construct
  misc_feature 1..375: note = Nucleotide sequence of hu1A5 VHH
  source 1..375: mol_type = other DNA
caggtccaattagtggaaagtggtgggggattagtgcaaccgggcggctccctccgcctttcctgcgccgcttctggcagaatcttctccaactactccgttggatggtttcgtcaggccccaggaaaagagagagaattcgtggctgctatcatatggagcacggggaccacctactatgccgatagcgtcaaaggcaggttcactatcagcagggataatagcaagaatacactatacttgcaaatgaactcgctgcgagccgaagacacagccgtctactactgtgcggcgtcatttaaatacagcggcatttacggccgagaggcagatttcggaagttgggggcagggaaccttggtgacagtctcctcg

SEQ ID NO: 41 - DNA, 45 bp, synthetic construct
  misc_feature 1..45: note = The nucleic acid sequence of linker
  source 1..45: mol_type = other DNA
ggaggcggaggttctggcggcggaggaagtggtggcggaggctct

SEQ ID NO: 42 - DNA, 711 bp, synthetic construct
  misc_feature 1..711: note = The nucleic acid sequence of the CAR non-antigen binding domain
  source 1..711: mol_type = other DNA
ttcgtccccgtgttcctgcctgccaagccaacaactacccctgctccacgaccacctactccagcacctaccatcgcaagtcagcccctgtcactgcgacctgaggcttgccggccagcagctggaggagcagtgcacacccgaggcctggacttcgcatgcgatatctacatttgggcaccactggctggaacctgtggggtcctgctgctgagcctggtcatcaccctgtattgtaaccacagaaataaaagggggcgcaagaaactgctgtacatcttcaagcagccttttatgcgcccagtgcagacaactcaggaggaagacggatgctcttgtcggttcccagaggaggaggaaggaggctgcgagctgagagtgaagttcagccggagcgccgatgcaccagcatatcagcagggacagaatcagctgtacaacgagctgaatctgggcaggcgcgaggaatatgacgtgctggataagcgacgaggacgggaccccgaaatgggaggaaaacccagaaggaagaaccctcaggaggggctgtataatgaactgcagaaagacaagatggctgaggcatacagcgaaattggaatgaaaggagagcgccgacgggggaagggacacgatgggctgtaccagggactgtcaaccgccactaaagatacctacgacgcactgcacatgcaggctctgcccccaaga

SEQ ID NO: 43 - DNA, 54 bp, synthetic construct
  misc_feature 1..54: note = The nucleic acid encoding the T2A peptide
  source 1..54: mol_type = other DNA
gagggcagaggcagcctgctgacatgtggcgacgtggaagagaaccctggcccc

SEQ ID NO: 44 - protein, 18 aa, synthetic construct
  REGION 1..18: note = T2A
EGRGSLLTCGDVEENPGP

SEQ ID NO: 45 - DNA, 612 bp, synthetic construct
  misc_feature 1..612: note = The nucleic acids encoding the 1st mIL-15
  source 1..612: mol_type = other DNA
atggccttaccagtgaccgccttgctcctgccgctggccttgctgctccacgccgccaggccgaactgggtgaatgtaataagtgatttgaaaaaaattgaagatcttattcaatctatgcatattgatgctactttatatacggaaagtgatgttcaccccagttgcaaagtaacagcaatgaagtgctttctcttggagttacaagttatttcacttgagtccggagatgcaagtattcatgatacagtagaaaatctgatcatcctagcaaacaacagtttgtcttctaatgggaatgtaacagaatctggatgcaaagaatgtgaggaactggaggaaaaaaatattaaagaatttttgcagagttttgtacatattgtccaaatgttcatcaacacttctaccacgacgccagcgccgcgaccaccaacaccggcgcccaccatcgcgtcgcagcccctgtccctgcgcccagaggcgtgccggccagcggcggggggcgcagtgcacacgagggggctggacttcgcctgtgatatctacatctgggcgcccttggccgggacttgtggggtccttctcctgtcactggttatcaccctttactgc

SEQ ID NO: 46 - protein, 204 aa, synthetic construct
  REGION 1..204: note = The 1st mIL-15
MALPVTALLLPLALLLHAARPNWVNVISDLKKIEDLIQSMHIDATLYTESDVHPSCKVTAMKCFLLELQVISLESGDASIHDTVENLIILANNSLSSNGNVTESGCKECEELEEKNIKEFLQSFVHIVQMFINTSTTTPAPRPPTPAPTIASQPLSLRPEACRPAAGGAVHTRGLDFACDIYIWAPLAGTCGVLLLSLVITLYC

SEQ ID NO: 47 - DNA, 404 bp, synthetic construct
  misc_feature 1..404: note = The nucleic acid encoding the extracellular domain of the 1st mIL-15
  source 1..404: mol_type = other DNA
atggccttaccagtgaccgccttgctcctgccgctggccttgctgctccacgccgccaggccgaactgggtgaatgtaataagtgatttgaaaaaaattgaagatcttattcaatctatgcatattgatgctactttatatacggaaagtgatgttcaccccagttgcaaagtaacagcaatgaagtgctttctcttggagttacaagttatttcacttgagtccggagatgcaagtattcatgatacagtagaaaatctgatcatcctagcaaacaacagtttgtcttctaatgggaatgtaacagaatctggatgcaaagaatgtgaggaactggaggaaaaaaatattaaagaatttttgcagagttttgtacatattgtccaaatgttcatcaacacttc

SEQ ID NO: 48 - protein, 135 aa, synthetic construct
  REGION 1..135: note = The amino acids in the extracellular domain of the 1st mIL-15
MALPVTALLLPLALLLHAARPNWVNVISDLKKIEDLIQSMHIDATLYTESDVHPSCKVTAMKCFLLELQVISLESGDASIHDTVENLIILANNSLSSNGNVTESGCKECEELEEKNIKEFLQSFVHIVQMFINTS

SEQ ID NO: 49 - DNA, 135 bp, synthetic construct
  misc_feature 1..135: note = The nucleic acids encoding the hinge region of the 1st mIL-15
  source 1..135: mol_type = other DNA
accacgacgccagcgccgcgaccaccaacaccggcgcccaccatcgcgtcgcagcccctgtccctgcgcccagaggcgtgccggccagcggcggggggcgcagtgcacacgagggggctggacttcgcctgtgat

SEQ ID NO: 50 - protein, 45 aa, synthetic construct
  REGION 1..45: note = The amino acids in the hinge region of the 1st mIL-15
TTTPAPRPPTPAPTIASQPLSLRPEACRPAAGGAVHTRGLDFACD

SEQ ID NO: 51 - DNA, 72 bp, synthetic construct
  misc_feature 1..72: note = The nucleic acids encoding the transmembrane domain of the 1st mIL-15
  source 1..72: mol_type = other DNA
atctacatctgggcgcccttggccgggacttgtggggtccttctcctgtcactggttatcaccctttactgc

SEQ ID NO: 52 - protein, 24 aa, synthetic construct
  REGION 1..24: note = The amino acids in the transmembrane domain of the 1st mIL-15
IYIWAPLAGTCGVLLLSLVITLYC

SEQ ID NO: 53 - DNA, 1185 bp, synthetic construct
  misc_feature 1..1185: note = The nucleic acids encoding the 2nd mIL-15
  source 1..1185: mol_type = other DNA
atggactggacgtggatcttgttcctggttgcagcagcaactcgtgtgcacagtaattgggtgaacgtcatcagcgatctgaaaaaaatagaagatctgattcagtccatgcatattgacgctacactctacacggagtccgacgtgcatccgtcctgcaaggtgaccgccatgaaatgtttcctgttggagctgcaggtcatcagcctcgagagcggagatgcttcaatacacgacaccgtcgagaatttgattattttggcaaataattccttgtcgtctaacggcaatgtcactgaaagcggttgcaaagagtgtgaagaattggaagaaaagaatatcaaggagtttctccagtcttttgttcatattgttcagatgttcatcaacacatcgagtggcggcggcagcggtggggggggttctggcggcggcggctccggaggtggtgggtccggtggaggtagtctgcagatcacttgtccacctcctatgtcagtggagcatgcggacatttgggtgaagagctacagtttatactcccgcgaaaggtacatctgcaatagcggattcaaacgcaaagcaggcacttcatcactcactgagtgtgtgttgaataaggcaaccaacgtggctcattggacaactccttccctgaagtgcattcgagaccccgccctcgtccatcagcgcccagccccaccttctacagtcaccaccgccggcgtgacacctcagcccgaaagccttagcccttccgggaaagaaccagctgcttctagcccctcatcaaacaataccgccgctactacagccgccattgtcccaggaagccagctgatgccgtccaagagccccagtactgggaccactgaaatctcctcccatgaaagctcccacgggactccgagtcagaccaccgcaaaaaattgggagctgactgctagcgcatcacaccagccccccggtgtgtatccacagggtcactctgatactacggttgctataagcacgagtactgtattactgtgcggtctgtccgccgtctctctgctggcctgctatctgaagtcccggcaaacacccccccttgcgtcagtggaaatggaagccatggaggcattgccggtgacgtggggaacttcatctagggacgaggacctggaaaactgtagccaccacctc

SEQ ID NO: 54 - protein, 395 aa, synthetic construct [sequence omitted]

SEQ ID NO: 55 - DNA, 396 bp, synthetic construct
  misc_feature 1..396: note = The nucleic acid encoding the extracellular domain of the 2nd mIL-15
  source 1..396: mol_type = other DNA
atggactggacgtggatcttgttcctggttgcagcagcaactcgtgtgcacagtaattgggtgaacgtcatcagcgatctgaaaaaaatagaagatctgattcagtccatgcatattgacgctacactctacacggagtccgacgtgcatccgtcctgcaaggtgaccgccatgaaatgtttcctgttggagctgcaggtcatcagcctcgagagcggagatgcttcaatacacgacaccgtcgagaatttgattattttggcaaataattccttgtcgtctaacggcaatgtcactgaaagcggttgcaaagagtgtgaagaattggaagaaaagaatatcaaggagtttctccagtcttttgttcatattgttcagatgttcatcaacacatcg

SEQ ID NO: 56 - protein, 132 aa, synthetic construct
  REGION 1..132: note = The amino acids in the extracellular domain of the 2nd mIL-15
MDWTWILFLVAAATRVHSNWVNVISDLKKIEDLIQSMHIDATLYTESDVHPSCKVTAMKCFLLELQVISLESGDASIHDTVENLIILANNSLSSNGNVTESGCKECEELEEKNIKEFLQSFVHIVQMFINTS

SEQ ID NO: 57 - DNA, 78 bp, synthetic construct
  misc_feature 1..78: note = The nucleic acids encoding the hinge region of the 2nd mIL-15
  source 1..78: mol_type = other DNA
agtggcggcggcagcggtggggggggttctggcggcggcggctccggaggtggtgggtccggtggaggtagtctgcag

SEQ ID NO: 58 - protein, 26 aa, synthetic construct
  REGION 1..26: note = The amino acids in the hinge region of the 2nd mIL-15
SGGGSGGGGSGGGGSGGGGSGGGSLQ

SEQ ID NO: 59 - DNA, 711 bp, synthetic construct
  misc_feature 1..711: note = The nucleic acids encoding the transmembrane domain of the 2nd mIL-15
  source 1..711: mol_type = other DNA
atcacttgtccacctcctatgtcagtggagcatgcggacatttgggtgaagagctacagtttatactcccgcgaaaggtacatctgcaatagcggattcaaacgcaaagcaggcacttcatcactcactgagtgtgtgttgaataaggcaaccaacgtggctcattggacaactccttccctgaagtgcattcgagaccccgccctcgtccatcagcgcccagccccaccttctacagtcaccaccgccggcgtgacacctcagcccgaaagccttagcccttccgggaaagaaccagctgcttctagcccctcatcaaacaataccgccgctactacagccgccattgtcccaggaagccagctgatgccgtccaagagccccagtactgggaccactgaaatctcctcccatgaaagctcccacgggactccgagtcagaccaccgcaaaaaattgggagctgactgctagcgcatcacaccagccccccggtgtgtatccacagggtcactctgatactacggttgctataagcacgagtactgtattactgtgcggtctgtccgccgtctctctgctggcctgctatctgaagtcccggcaaacacccccccttgcgtcagtggaaatggaagccatggaggcattgccggtgacgtggggaacttcatctagggacgaggacctggaaaactgtagccaccacctc

SEQ ID NO: 60 - protein, 237 aa, synthetic construct
  REGION 1..237: note = The amino acids in the transmembrane domain of the 2nd mIL-15
ITCPPPMSVEHADIWVKSYSLYSRERYICNSGFKRKAGTSSLTECVLNKATNVAHWTTPSLKCIRDPALVHQRPAPPSTVTTAGVTPQPESLSPSGKEPAASSPSSNNTAATTAAIVPGSQLMPSKSPSTGTTEISSHESSHGTPSQTTAKNWELTASASHQPPGVYPQGHSDTTVAISTSTVLLCGLSAVSLLACYLKSRQTPPLASVEMEAMEALPVTWGTSSRDEDLENCSHHL

SEQ ID NO: 61 - DNA, 63 bp, synthetic construct
  misc_feature 1..63: note = The nucleic acid sequence of CD8A signal peptide
  source 1..63: mol_type = other DNA
atggccttaccagtgaccgccttgctcctgccgctggccttgctgctccacgccgccaggccg

SEQ ID NO: 62 - protein, 21 aa, synthetic construct
  REGION 1..21: note = CD8A transmembrane domain
IYIWAPLAGTCGVLLLSLVIT

SEQ ID NO: 63 - protein, 21 aa, synthetic construct
  REGION 1..21: note = CD8B transmembrane domain
ITLGLLVAGVLVLLVSLGVAI

SEQ ID NO: 64 - protein, 27 aa, synthetic construct
  REGION 1..27: note = CD28 transmembrane domain
FWVLVVVGGVLACYSLLVTVAFIIFWV

SEQ ID NO: 65 - protein, 27 aa, synthetic construct
  REGION 1..27: note = 4-1BB transmembrane domain
IISFFLALTSTALLFLLFFLTLRFSVV

SEQ ID NO: 66 - protein, 22 aa, synthetic construct
  REGION 1..22: note = CD4 transmembrane domain
MALIVLGGVAGLLLFIGLGIFF

SEQ ID NO: 67 - protein, 21 aa, synthetic construct
  REGION 1..21: note = CD27 transmembrane domain
ILVIFSGMFLVFTLAGALFLH

SEQ ID NO: 68 - protein, 21 aa, synthetic construct
  REGION 1..21: note = CD7 transmembrane domain
AALAVISFLLGLGLGVACVLA

SEQ ID NO: 69 - protein, 21 aa, synthetic construct
  REGION 1..21: note = PD-1 transmembrane domain
VGVVGGLLGSLVLLVWVLAVI

SEQ ID NO: 70 - protein, 23 aa, synthetic construct
  REGION 1..23: note = TRAC transmembrane domain
VIGFRILLLKVAGFNLLMTLRLW

SEQ ID NO: 71 - protein, 21 aa, synthetic construct
  REGION 1..21: note = TRBC transmembrane domain
ILLGKATLYAVLVSALVLMAM

SEQ ID NO: 72 - protein, 26 aa, synthetic construct
  REGION 1..26: note = CD3 transmembrane domain
VMSVATIVIVDICITGGLLLLVYYWS

SEQ ID NO: 73 - protein, 21 aa, synthetic construct
  REGION 1..21: note = CD3 transmembrane domain
LCYLLDGILFIYGVILTALFL

SEQ ID NO: 74 - protein, 21 aa, synthetic construct
  REGION 1..21: note = CTLA-4 transmembrane domain
FLLWILAAVSSGLFFYSFLLT

SEQ ID NO: 75 - protein, 21 aa, synthetic construct
  REGION 1..21: note = LAG-3 transmembrane domain
LLFLILGVLSLLLLVTGAFGF

SEQ ID NO: 76 - protein, 30 aa, synthetic construct
  REGION 1..30: note = CD5 transmembrane domain
AGLAAGTVASIILALVLLVVLLVVCGPLAY

SEQ ID NO: 77 - protein, 21 aa, synthetic construct
  REGION 1..21: note = ICOS transmembrane domain
FWLPIGCAAFVVVCILGCILI

SEQ ID NO: 78 - protein, 21 aa, synthetic construct
  REGION 1..21: note = OX40 transmembrane domain
VAAILGLGLVLGLLGPLAILL

SEQ ID NO: 79 - protein, 21 aa, synthetic construct
  REGION 1..21: note = NKG2D transmembrane domain
PFFFCCFIAVAMGIRFIIMVA

SEQ ID NO: 80 - protein, 21 aa, synthetic construct
  REGION 1..21: note = 2B4 transmembrane domain
FLVIIVILSALFLGTLACFCV

SEQ ID NO: 81 - protein, 21 aa, synthetic construct
  REGION 1..21: note = FcRI transmembrane domain
LCYILDAILFLYGIVLTLLYC

SEQ ID NO: 82 - protein, 21 aa, synthetic construct
  REGION 1..21: note = BTLA transmembrane domain
LLPLGGLPLLITTCFCLFCCL

SEQ ID NO: 83 - protein, 21 aa, synthetic construct
  REGION 1..21: note = CD30 transmembrane domain
PVLFWVILVLVVVVGSSAFLL

SEQ ID NO: 84 - protein, 21 aa, synthetic construct
  REGION 1..21: note = GITR transmembrane domain
LGWLTVVLLAVAACVLLLTSA

SEQ ID NO: 85 - protein, 21 aa, synthetic construct
  REGION 1..21: note = HVEM transmembrane domain
WWFLSGSLVIVIVCSTVGLII

SEQ ID NO: 86 - protein, 21 aa, synthetic construct
  REGION 1..21: note = DAP10 transmembrane domain
LLAGLVAADAVASLLIVGAVF

SEQ ID NO: 87 - protein, 26 aa, synthetic construct
  REGION 1..26: note = CD2 transmembrane domain
IYLIIGICGGGSLLMVFVALLVFYIT

SEQ ID NO: 88 - protein, 23 aa, synthetic construct
  REGION 1..23: note = NKG2C transmembrane domain
LTAEVLGIICIVLMATVLKTIVL

SEQ ID NO: 89 - protein, 21 aa, synthetic construct
  REGION 1..21: note = LIGHT transmembrane domain
VGLGLLLLLMGAGLAVQGWFL

SEQ ID NO: 90 - protein, 21 aa, synthetic construct
  REGION 1..21: note = DAP12 transmembrane domain
GVLAGIVMGDLVLTVLIALAV

SEQ ID NO: 91 - protein, 24 aa, synthetic construct
  REGION 1..24: note = CD40L transmembrane domain
IFMYLLTVFLITQMIGSALFAVYL

SEQ ID NO: 92 - protein, 21 aa, synthetic construct
  REGION 1..21: note = TIM1 transmembrane domain
IYAGVCISVLVLLALLGVIIA

SEQ ID NO: 93 - protein, 21 aa, synthetic construct
  REGION 1..21: note = CD226 transmembrane domain
GGTVLLLLFVISITTIIVIFL

SEQ ID NO: 94 - protein, 21 aa, synthetic construct
  REGION 1..21: note = DR3 transmembrane domain
MFWVQVLLAGLVVPLLLGATL

SEQ ID NO: 95 - protein, 21 aa, synthetic construct
  REGION 1..21: note = CD45 transmembrane domain
ALIAFLAFLIIVTSIALLVVL

SEQ ID NO: 96 - protein, 21 aa, synthetic construct
  REGION 1..21: note = CD80 transmembrane domain
LLPSWAITLISVNGIFVICCL

SEQ ID NO: 97 - protein, 21 aa, synthetic construct
  REGION 1..21: note = CD86 transmembrane domain
WITAVLPTVIICVMVFCLILW

SEQ ID NO: 98 - protein, 21 aa, synthetic construct
  REGION 1..21: note = CD9 transmembrane domain1
LLFGFNFIFWLAGIAVLAIGL

SEQ ID NO: 99 - protein, 21 aa, synthetic construct
  REGION 1..21: note = CD9 transmembrane domain2
FYTGVYILIGAGALMMLVGFL

SEQ ID NO: 100 - protein, 24 aa, synthetic construct
  REGION 1..24: note = CD9 transmembrane domain3
MLGLFFGFLLVIFAIEIAAAIWGY

SEQ ID NO: 101 - protein, 26 aa, synthetic construct
  REGION 1..26: note = CD9 transmembrane domain4
IGAVGIGIAVVMIFGMIFSMILCCAI

SEQ ID NO: 102 - protein, 21 aa, synthetic construct
  REGION 1..21: note = CD16 transmembrane domain
VSFCLVMVLLFAVDTGLYFSV

SEQ ID NO: 103 - protein, 19 aa, synthetic construct
  REGION 1..19: note = CD22 transmembrane domain
VAVGLGSCLAILILAICGL

SEQ ID NO: 104 - protein, 23 aa, synthetic construct
  REGION 1..23: note = CD33 transmembrane domain
GAIGGAGVTALLALCLCLIFFIV

SEQ ID NO: 105 - protein, 21 aa, synthetic construct
  REGION 1..21: note = CD37 transmembrane domain1
FNLFFFVLGSLIFCFGIWILI

SEQ ID NO: 106 - protein, 15 aa, synthetic construct
  REGION 1..15: note = CD37 transmembrane domain2
VLAISGIFTMGIALL

SEQ ID NO: 107 - protein, 26 aa, synthetic construct
  REGION 1..26: note = CD37 transmembrane domain3
LLGLYFGMLLLLFATQITLGILISTQ

SEQ ID NO: 108 - protein, 25 aa, synthetic construct
  REGION 1..25: note = CD37 transmembrane domain4
LISIVGICLGVGLLELGFMTLSIFL

SEQ ID NO: 109 - protein, 21 aa, synthetic construct
  REGION 1..21: note = CD64 transmembrane domain
VLFYLAVGIMFLVNTVLWVTI

SEQ ID NO: 110 - protein, 21 aa, synthetic construct
  REGION 1..21: note = SLAM transmembrane domain
WAVYAGLLGGVIMILIMVVIL

SEQ ID NO: 111 - protein, 41 aa, synthetic construct
  REGION 1..41: note = CD28 intracellular co-stimulatory signaling domain
RSKRSRLLHSDYMNMTPRRPGPTRKHYQPYAPPRDFAAYRS

SEQ ID NO: 112 - protein, 42 aa, synthetic construct
  REGION 1..42: note = CD137 intracellular co-stimulatory signaling domain
KRGRKKLLYIFKQPFMRPVQTTQEEDGCSCRFPEEEEGGCEL

SEQ ID NO: 113 - protein, 48 aa, synthetic construct
  REGION 1..48: note = CD27 intracellular co-stimulatory signaling domain
QRRKYRSNKGESPVEPAEPCHYSCPREEEGSTIPIQEDYRKPEPACSP

SEQ ID NO: 114 - protein, 116 aa, synthetic construct
  REGION 1..116: note = CD2 intracellular co-stimulatory signaling domain
KRKKQRSRRNDEELETRAHRVATEERGRKPHQIPASTPQNPATSQHPPPPPGHRSQAPSHRPPPPGHRVQHQPQKRPPAPSGTQVHQQKGPPLPRPRVQPKPPHGAAENSLSPSSN

SEQ ID NO: 115 - protein, 39 aa, synthetic construct
  REGION 1..39: note = CD7 intracellular co-stimulatory signaling domain
RTQIKKLCSWRDKNSAACVVYEDMSHSRCNTLSSPNQYQ

SEQ ID NO: 116 - protein, 32 aa, synthetic construct
  REGION 1..32: note = CD8A intracellular co-stimulatory signaling domain
LYCNHRNRRRVCKCPRPVVKSGDKPSLSARYV

SEQ ID NO: 117 - protein, 19 aa, synthetic construct
  REGION 1..19: note = CD8B intracellular co-stimulatory signaling domain
HLCCRRRRARLRFMKQFYK

SEQ ID NO: 118 - protein, 42 aa, synthetic construct
  REGION 1..42: note = OX40 intracellular co-stimulatory signaling domain
ALYLLRRDQRLPPDAHKPPGGGSFRTPIQEEQADAHSTLAKI

SEQ ID NO: 119 - protein, 61 aa, synthetic construct
  REGION 1..61: note = CD226 intracellular co-stimulatory signaling domain
NRRRRRERRDLFTESWDTQKAPNNYRSPISTSQPTNQSMDDTREDIYVNYPTFSRRPKTRV

SEQ ID NO: 120 - protein, 197 aa, synthetic construct
  REGION 1..197: note = DR3 intracellular co-stimulatory signaling domain
TYTYRHCWPHKPLVTADEAGMEALTPPPATHLSPLDSAHTLLAPPDSSEKICTVQLVGNSWTPGYPETQEALCPQVTWSWDQLPSRALGPAAAPTLSPESPAGSPAMMLQPGPQLYDVMDAVPARRWKEFVRTLGLREAEIEAVEVEIGRFRDQQYEMLKRWRQQQPAGLGAVYAALERMGLDGCVEDLRSRLQRGP

SEQ ID NO: 121 - protein, 77 aa, synthetic construct
  REGION 1..77: note = SLAM intracellular co-stimulatory signaling domain
QLRRRGKTNHYQTTVEKKSLTIYAQVQKPGPLQKKLDSFPAQDPCTTIYVAATEPVPESVQETNSITVYASVTLPES

SEQ ID NO: 122 - protein, 29 aa, synthetic construct
  REGION 1..29: note = ICAM-1 intracellular co-stimulatory signaling domain
NRQRKIKKYRLQQAQKGTPMKPNTQATPP

SEQ ID NO: 123 - protein, 51 aa, synthetic construct
  REGION 1..51: note = NKG2D intracellular co-stimulatory signaling domain
MGWIRGRRSRHSWEMSEFHNYNLDLKKSDFSTRWQKQRCPVVKSKCRENAS

SEQ ID NO: 124 - protein, 70 aa, synthetic construct
  REGION 1..70: note = NKG2C intracellular co-stimulatory signaling domain
MSKQRGTFSEVSLAQDPKRQQRKPKGNKSSISGTEQEIFQVELNLQNPSLNHQGIDKIYDCQGLLPPPEK

SEQ ID NO: 125 - protein, 47 aa, synthetic construct
  REGION 1..47: note = B7-H3 intracellular co-stimulatory signaling domain
CWRKIKQSCEEENAGAEDQDGEGEGSKTALQPLKHSDSKEDDGQEIA

SEQ ID NO: 126 - protein, 120 aa, synthetic construct
  REGION 1..120: note = 2B4 intracellular co-stimulatory signaling domain
WRRKRKEKQSETSPKEFLTIYEDVKDLKTRRNHEQEQTFPGGGSTIYSMIQSQSSAPTSQEPAYTLYSLIQPSRKSGSRKRNHSPSFNSTIYEVIGKSQPKAQNPARLSRKELENFDVYS

SEQ ID NO: 127 - protein, 42 aa, synthetic construct
  REGION 1..42: note = FcRI intracellular co-stimulatory signaling domainFcRI intracellular signaling domain
RLKIQVRKAAITSYEKSDGVYTGLSTRNQETYETLKHEKPPQ

SEQ ID NO: 128 - protein, 111 aa, synthetic construct
  REGION 1..111: note = BTLA intracellular co-stimulatory signaling domain
RRHQGKQNELSDTAGREINLVDAHLKSEQTEASTRQNSQVLLSETGIYDNDPDLCFRMQEGSEVYSNPCLEENKPGIVYASLNHSVIGPNSRLARNVKEAPTEYASICVRS

SEQ ID NO: 129 - protein, 58 aa, synthetic construct
  REGION 1..58: note = GITR intracellular co-stimulatory signaling domain
QLGLHIWQLRSQCMWPRETQLLLEVPPSTEDARSCQFPEEERGERSAEEKGRLGDLWV

SEQ ID NO: 130 - protein, 60 aa, synthetic construct
  REGION 1..60: note = HVEM intracellular co-stimulatory signaling domain
CVKRRKPRGDVVKVIVSVQRKRQEAEGEATVIEALQAPPDVTTVAVEETIPSFTGRSPNH

SEQ ID NO: 131 - protein, 24 aa, synthetic construct
  REGION 1..24: note = DAP10 intracellular co-stimulatory signaling domainDAP10 intracellular signaling domain
LCARPRRSPAQEDGKVYINMPGRG

SEQ ID NO: 132 - protein, 52 aa, synthetic construct
  REGION 1..52: note = DAP12 intracellular co-stimulatory signaling domainDAP-12 intracellular signaling domain
YFLGRLVPRGRGAAEAATRKQRITETESPYQELQGQRSDVYSDLNTQRPYYK

SEQ ID NO: 133 - protein, 189 aa, synthetic construct
  REGION 1..189: note = CD30 intracellular co-stimulatory signaling domain
CHRRACRKRIRQKLHLCYPVQTSQPKLELVDSRPRRSSTQLRSGASVTEPVAEERGLMSQPLMETCHSVGAAYLESLPLQDASPAGGPSSPRDLPEPRVSTEHTNNKIEKIYIMKADTVIVGTVKAELPEGRGLAGPAEPELEEELEADHTPHYPEQETEPPLGSCSDVMLSVEEEGKEDPLPTAASGK

SEQ ID NO: 134 - protein, 62 aa, synthetic construct
  REGION 1..62: note = CD40 intracellular co-stimulatory signaling domain
KKVAKKPTNKAPHPKQEPQEINFPDDLPGSNTAAPVQETLHGCQPVTQEDGKESRISVQERQ

SEQ ID NO: 135 - protein, 22 aa, synthetic construct
  REGION 1..22: note = CD40L intracellular co-stimulatory signaling domain
MIETYNQTSPRSAATGLPISMK

SEQ ID NO: 136 - protein, 48 aa, synthetic construct
  REGION 1..48: note = TIM1 intracellular co-stimulatory signaling domain
KKYFFKKEVQQLSVSFSSLQIKALQNAVEKEVQAEDNIYIENSLYATD

SEQ ID NO: 137 - protein, 97 aa, synthetic construct
  REGION 1..97: note = PD-1 intracellular co-stimulatory signaling domain
CSRAARGTIGARRTGQPLKEDPSAVPVFSVDYGELDFQWREKTPEPPVPCVPEQTEYATIVFPSGMGTSSPARRGSADGPRSAQPLRPEDGHCSWPL

SEQ ID NO: 138 - protein, 59 aa, synthetic construct
  REGION 1..59: note = LFA-1 intracellular co-stimulatory signaling domain
YKVGFFKRNLKEKMEAGRGVPNGIPAEDSEQLASGQEAGDPGCLKPLHEKDSESGGGKD

SEQ ID NO: 139 - protein, 182 aa, synthetic construct
  REGION 1..182: note = LIGHT intracellular co-stimulatory signaling domain
LQLHWRLGEMVTRLPDGPAGSWEQLIQERRSHEVNPAAHLTGANSSLTGSGGPLLWETQLGLAFLRGLSYHDGALVVTKAGYYYIYSKVQLGGVGCPLGLASTITHGLYKRTPRYPEELELLVSQQSPCGRATSSSRVWWDSSFLGGVVHLEAGEKVVVRVLDERLVRLRDGTRSYFGAFMV

SEQ ID NO: 140 - protein, 98 aa, synthetic construct
  REGION 1..98: note = JAML intracellular co-stimulatory signaling domain
KKTCGNKSSVNSTVLVKNTKKTNPEIKEKPCHFERCEGEKHIYSPIIVREVIEEEEPSEKSEATYMTMHPVWPSLRSDRNNSLEKKSGGGMPKTQQAF

SEQ ID NO: 141 - protein, 107 aa, synthetic construct
  REGION 1..107: note = CD100 intracellular co-stimulatory signaling domain
YKGYLPRQCLKFRSALLIGKKKPKSDFCDREQSLKETLVEPGSFSQQNGEHPKPALDTGYETEQDTITSKVPTDREDSQRIDDLSARDKPFDVKCELKFADSDADGD

SEQ ID NO: 142 - protein, 38 aa, synthetic construct
  REGION 1..38: note = ICOS intracellular co-stimulatory signaling domain
CWLTKKKYSSSVHDPNGEYMFMRAVNTAKKSRLTDVTL

SEQ ID NO: 143 - protein, 296 aa, synthetic construct
  REGION 1..296: note = MyD88 intracellular co-stimulatory signaling domain
MAAGGPGAGSAAPVSSTSSLPLAALNMRVRRRLSLFLNVRTQVAADWTALAEEMDFEYLEIRQLETQADPTGRLLDAWQGRPGASVGRLLELLTKLGRDDVLLELGPSIEEDCQKYILKQQQEEAEKPLQVAAVDSSVPRTAELAGITTLDDPLGHMPERFDAFICYCPSDIQFVQEMIRQLEQTNYRLKLCVSDRDVLPGTCVWSIASELIEKRCRRMVVVVSDDYLQSKECDFQTKFALSLSPGAHQKRLIPIKYKAMKKEFPSILRFITVCDYTNPCTKSWFWTRLAKALSLP

SEQ ID NO: 144 - protein, 113 aa, synthetic construct
  REGION 1..113: note = CD3 intracellular signaling domain
RVKFSRSADAPAYQQGQNQLYNELNLGRREEYDVLDKRRGRDPEMGGKPQRRKNPQEGLYNELQKDKMAEAYSEIGMKGERRRGKGHDGLYQGLSTATKDTYDALHMQALPPR

SEQ ID NO: 145 - protein, 45 aa, synthetic construct
  REGION 1..45: note = CD3 intracellular signaling domain
GHETGRLSGAADTQALLRNDQVYQPLRDRDDAQYSHLGGNWARNK

SEQ ID NO: 146 - protein, 45 aa, synthetic construct
  REGION 1..45: note = CD3 intracellular signaling domain
GQDGVRQSRASDKQTLLPNDQLYQPLKDREDDQYSHLQGNQLRRN

SEQ ID NO: 147 - protein, 55 aa, synthetic construct
  REGION 1..55: note = CD3 intracellular signaling domain
KNRKAKAKPVTRGAGAGGRQRGQNKERPPPVPNPDYEPIRKGQRDLYSGLNQRRI

SEQ ID NO: 148 - protein, 61 aa, synthetic construct
  REGION 1..61: note = CD79a intracellular signaling domain
RKRWQNEKLGLDAGDEYEDENLYEGLNLDDCSMYEDISRGLQGTYQDVGSLNIGDVQLEKP

SEQ ID NO: 149 - protein, 49 aa, synthetic construct
  REGION 1..49: note = CD79b intracellular signaling domain
LDKDDSKAGMEEDHTYEGLDIDQTATYEDIVTLRTGEVKWSVGEHPGQE

SEQ ID NO: 150 - protein, 44 aa, synthetic construct
  REGION 1..44: note = FceRI intracellular signaling domain
ICGAGEELKGNKVPEDRVYEELNIYSATYSELEDPGEMSPPIDL

SEQ ID NO: 151 - protein, 77 aa, synthetic construct
  REGION 1..77: note = FcRIIa intracellular signaling domain
CRKKRISANSTDPVKAAQFEPPGRQMIAIRKRQLEETNNDYETADGGYMTLNPRAPTDDDKNIYLTLPPNDHVNSNN

SEQ ID NO: 152 - protein, 58 aa, synthetic construct
  REGION 1..58: note = BLV gp30 intracellular signaling domain
KCLTSRLLKLLRQAPHFPEISFPPKPDSDYQALLPSAPEIYSHLSPTKPDYINLRPCP

SEQ ID NO: 153 - protein, 123 aa, synthetic construct
  REGION 1..123: note = EBV LMP2A intracellular signaling domain
MGSLEMVPMGAGPPSPGGDPDGYDGGNNSQYPSASGSSGNTPTPPNDEERESNEEPPPPYEDPYWGNGDRHSDYQPLGTQDQSLYLGLQHDGNDGLPPPPYSPRDDSSQHIYEEAGRGSMNPV

SEQ ID NO: 154 - protein, 260 aa, synthetic construct
  REGION 1..260: note = SIV PBj14 Nef intracellular signaling domain
GGVTSKKQRRRGGNLYERLLQARGETYGRLWEGLEGEYSQSQDASGKGLSSLSCEPQKYCEGQFMNTPWRNPATERAKLDYRQQNMDDVDSADLVGCPVSPRVPVRIMTYKLAIDMSHFIKEKGGLEGIYYSDRRHKILDLYLEKEEGIIPDWQNYTAGPGIRYPMFFGWLWKLVPVNVSDEAQEDETHYLMHPAQTSQWDDPWGEVLAWKFDPKLAYNYKAFVEHPEEFGSQSGLSKEEVQRRLTARGLLKMADKKKTS

SEQ ID NO: 155 - protein, 134 aa, synthetic construct
  REGION 1..134: note = CD28 hinge region
NKILVKQSPMLVAYDNAVNLSCKYSYNLFSREFRASLHKGLDSAVEVCVVYGNYSQQLQVYSKTGFNCDGKLGNESVTFYLQNLYVNQTDIYFCKIEVMYPPPYLDNEKSNGTIIHVKGKHLCPSPLFPGPSKP

SEQ ID NO: 156 - protein, 220 aa, synthetic construct
  REGION 1..220: note = IgG1 hinge region
PCPAPELLGGPSVFLFPPKPKDTLMISRTPEVTCVVVDVSHEDPEVKFNWYVDGVEVHNAKTKPREEQYNSTYRVVSVLTVLHQDWLNGKEYKCKVSNKALPAPIEKTISKAKGQPREPQVYTLPPSRDELTKNQVSLTCLVKGFYPSDIAVEWESNGQPENNYKTTPPVLDSDGSFFLYSKLTVDKSRWQQGNVFSCSVMHEALHNHYTQKSLSLSPGK

SEQ ID NO: 157 - protein, 217 aa, synthetic construct
  REGION 1..217: note = IgG4 hinge region
APEFLGGPSVFLFPPKPKDTLMISRTPEVTCVVVDVSQEDPEVQFNWYVDGVEVHNAKTKPREEQFNSTYRVVSVLTVLHQDWLNGKEYKCKVSNKGLPSSIEKTISKAKGQPREPQVYTLPPSQEEMTKNQVSLTCLVKGFYPSDIAVEWESNGQPENNYKTTPPVLDSDGSFFLYSRLTVDKSRWQEGNVFSCSVMHEALHNHYTQKSLSLSLGK

SEQ ID NO: 158 - protein, 223 aa, synthetic construct
  REGION 1..223: note = IgD hinge region
CPSHTQPLGVYLLTPAVQDLWLRDKATFTCFVVGSDLKDAHLTWEVAGKVPTGGVEEGLLERHSNGSQSQHSRLTLPRSLWNAGTSVTCTLNHPSLPPQRLMALREPAQAPVKLSLNLLASSDPPEAASWLLCEVSGFSPPNILLMWLEDQREVNTSGFAPARPPPQPRSTTFWAWSVLRVPAPPSPQPATYTCVVSHEDSRTLLNASRSLEVSYVTDHGPMK

SEQ ID NO: 159 - protein, 163 aa, synthetic construct
  REGION 1..163: note = 4-1BB hinge region
LQDPCSNCPAGTFCDNNRNQICSPCPPNSFSSAGGQRTCDICRQCKGVFRTRKECSSTSNAECDCTPGFHCLGAGCSMCEQDCKQGQELTKKGCKDCCFGTFNDQKRGICRPWTNCSLDGKSVLVNGTKERDVVCGPSPADLSPGASSVTPPAPAREPGHSPQ

SEQ ID NO: 160 - protein, 371 aa, synthetic construct
  REGION 1..371: note = CD4 hinge region
KKVVLGKKGDTVELTCTASQKKSIQFHWKNSNQIKILGNQGSFLTKGPSKLNDRADSRRSLWDQGNFPLIIKNLKIEDSDTYICEVEDQKEEVQLLVFGLTANSDTHLLQGQSLTLTLESPPGSSPSVQCRSPRGKNIQGGKTLSVSQLELQDSGTWTCTVLQNQKKVEFKIDIVVLAFQKASSIVYKKEGEQVEFSFPLAFTVEKLTGSGELWWQAERASSSKSWITFDLKNKEVSVKRVTQDPKLQMGKKLPLHLTLPQALPQYAGSGNLTLALEAKTGKLHQEVNLVVMRATQLQKNLTCEVWGPTSPKLMLSLKLENKEAKVSKREKAVWVLNPEAGMWQCLLSDSGQVLLESNIKVLPTWSTPVQP

SEQ ID NO: 161 - protein, 172 aa, synthetic construct
  REGION 1..172: note = CD27 hinge region
ATPAPKSCPERHYWAQGKLCCQMCEPGTFLVKDCDQHRKAAQCDPCIPGVSFSPDHHTRPHCESCRHCNSGLLVRNCTITANAECACRNGWQCRDKECTECDPLPNPSLTARSSQALSPHPQPTHLPYVSEMLEARTAGHMQTLADFRQLPARTLSTHWPPQRSLCSSDFIR

SEQ ID NO: 162 - protein, 155 aa, synthetic construct
  REGION 1..155: note = CD7 hinge region
AQEVQQSPHCTTVPVGASVNITCSTSGGLRGIYLRQLGPQPQDIIYYEDGVVPTTDRRFRGRIDFSGSQDNLTITMHRLQLSDTGTYTCQAITEVNVYGSGTLVLVTEEQSQGWHRCSDAPPRASALPAPPTGSALPDPQTASALPDPPAASALP

SEQ ID NO: 163 - protein, 161 aa, synthetic construct
  REGION 1..161: note = CD8A hinge region
SQFRVSPLDRTWNLGETVELKCQVLLSNPTSGCSWLFQPRGAAASPTFLLYLSQNKPKAAEGLDTQRFSGKRLGDTFVLTLSDFRRENEGYYFCSALSNSIMYFSHFVPVFLPAKPTTTPAPRPPTPAPTIASQPLSLRPEACRPAAGGAVHTRGLDFACD

SEQ ID NO: 164 - protein, 147 aa, synthetic construct
  REGION 1..147: note = PD-1 hinge region
FLDSPDRPWNPPTFSPALLVVTEGDNATFTCSFSNTSESFVLNWYRMSPSNQTDKLAAFPEDRSQPGQDCRFRVTQLPNGRDFHMSVVRARRNDSGTYLCGAISLAPKAQIKESLRAELRVTERRAEVPTAHPSPSPRPAGQFQTLV

SEQ ID NO: 165 - protein, 120 aa, synthetic construct
  REGION 1..120: note = ICOS hinge region
EINGSANYEMFIFHNGGVQILCKYPDIVQQFKMQLLKGGQILCDLTKTKGSGNTVSIKSLKFCHSQLSNNSVSFFLYNLDHSHANYYFCNLSIFDPPPFKVTLTGGYLHIYESQLCCQLK

SEQ ID NO: 166 - protein, 133 aa, synthetic construct
  REGION 1..133: note = OX40 hinge region
QVSHRYPRIQSIKVQFTEYKKEKGFILTSQKEDEIMKVQNNSVIINCDGFYLISLKGYFSQEVNISLHYQKDEEPLFQLKKVRSVNSLMVASLTYKDKVYLNVTTDNTSLDDFHVNGGELILIHQNPGEFCVL

SEQ ID NO: 167 - protein, 144 aa, synthetic construct
  REGION 1..144: note = NKG2D hinge region
IWSAVFLNSLFNQEVQIPLTESYCGPCPKNWICYKNNCYQFFDESKNWYESQASCMSQNASLLKVYSKEDQDLLKLVKSYHWMGLVHIPTNGSWQWEDGSILSPNLLTIIEMQKGDCALYASSFKGYIENCSTPNTYICMQRTV

SEQ ID NO: 168 - protein, 138 aa, synthetic construct
  REGION 1..138: note = NKG2C hinge region
IPFLEQNNSSPNTRTQKARHCGHCPEEWITYSNSCYYIGKERRTWEESLLACTSKNSSLLSIDNEEEMKFLASILPSSWIGVFRNSSHHPWVTINGLAFKHKIKDSDNAELNCAVLQVNRLKSAQCGSSMIYHCKHKL

SEQ ID NO: 169 - protein, 5 aa, synthetic construct
  REGION 1..5: note = FcRI hinge region
LGEPQ

SEQ ID NO: 170 - protein, 127 aa, synthetic construct
  REGION 1..127: note = BTLA hinge region
KESCDVQLYIKRQSEHSILAGDPFELECPVKYCANRPHVTWCKLNGTTCVKLEDRQTSWKEEKNISFFILHFEPVLPNDNGSYRCSANFQSNLIESHSTTLYVTDVKSASERPSKDEMASRPWLLYR

SEQ ID NO: 171 - protein, 137 aa, synthetic construct
  REGION 1..137: note = GITR hinge region
QRPTGGPGCGPGRLLLGTGTDARCCRVHTTRCCRDYPGEECCSEWDCMCVQPEFHCGDPCCTTCRHHPCPPGQGVQSQGKFSFGFQCIDCASGTFSGGHEGHCKPWTDCTQFGFLTVFPGNKTHNAVCVPGSPPAEP

SEQ ID NO: 172 - protein, 30 aa, synthetic construct
  REGION 1..30: note = DAP10 hinge region
QTTPGERSSLPAFYPGTSGSCSGCGSLSLP

SEQ ID NO: 173 - protein, 275 aa, synthetic construct
  REGION 1..275: note = TIM1 hinge region
SVKVGGEAGPSVTLPCHYSGAVTSMCWNRGSCSLFTCQNGIVWTNGTHVTYRKDTRYKLLGDLSRRDVSLTIENTAVSDSGVYCCRVEHRGWFNDMKITVSLEIVPPKVTTTPIVTTVPTVTTVRTSTTVPTTTTVPMTTVPTTTVPTTMSIPTTTTVLTTMTVSTTTSVPTTTSIPTTTSVPVTTTVSTFVPPMPLPRQNHEPVATSPSSPQPAETHPTTLQGAIRREPTSSPLYSYTTDGNDTVTESSDGLWNNNQTQLFLEHSLLTANTTKG

SEQ ID NO: 174 - protein, 217 aa, synthetic construct
  REGION 1..217: note = SLAM hinge region
ASYGTGGRMMNCPKILRQLGSKVLLPLTYERINKSMNKSIHIVVTMAKSLENSVENKIVSLDPSEAGPPRYLGDRYKFYLENLTLGIRESRKEDEGWYLMTLEKNVSVQRFCLQLRLYEQVSTPEIKVLNKTQENGTCTLILGCTVEKGDHVAYSWSEKAGTHPLNPANSSHLLSLTLGPQHADNIYICTVSNPISNNSQTFSPWPGCRTDPSETKP

SEQ ID NO: 175 - protein, 367 aa, synthetic construct
  REGION 1..367: note = CD30 hinge region
FPQDRPFEDTCHGNPSHYYDKAVRRCCYRCPMGLFPTQQCPQRPTDCRKQCEPDYYLDEADRCTACVTCSRDDLVEKTPCAWNSSRVCECRPGMFCSTSAVNSCARCFFHSVCPAGMIVKFPGTAQKNTVCEPASPGVSPACASPENCKEPSSGTIPQAKPTPVSPATSSASTMPVRGGTRLAQEAASKLTRAPDSPSSVGRPSSDPGLSPTQPCPEGSGDCRKQCEPDYYLDEAGRCTACVSCSRDDLVEKTPCAWNSSRTCECRPGMICATSATNSCARCVPYPICAAETVTKPQDMAEKDTTFEAPPLGTQPDCNPTPENGEAPASTSPTQSLLVDSQASKTLPIPTSAPVALSSTGKPVLDAG

SEQ ID NO: 176 - protein, 37 aa, synthetic construct
  REGION 1..37: note = LIGHT hinge region
MEESVVRPSVFVVDGQTDIPFTRLGRSHRRQSCSVAR

SEQ ID NO: 177 - RNA, 20 nt, synthetic construct
  modified_base 5: mod_base = OTHER; note = thymine
  modified_base 7: mod_base = OTHER; note = thymine
  modified_base 9: mod_base = OTHER; note = thymine
  modified_base 14: mod_base = OTHER; note = thymine
  modified_base 17: mod_base = OTHER; note = thymine
  misc_feature 1..20: note = TRAC sg9
  source 1..20: mol_type = other RNA
agagtctctcagctggtaca

SEQ ID NO: 178 - RNA, 20 nt, synthetic construct
  modified_base 1: mod_base = OTHER; note = thymine
  modified_base 3: mod_base = OTHER; note = thymine
  modified_base 6: mod_base = OTHER; note = thymine
  modified_base 12: mod_base = OTHER; note = thymine
  modified_base 17: mod_base = OTHER; note = thymine
  modified_base 19: mod_base = OTHER; note = thymine
  misc_feature 1..20: note = TRAC sg10
  source 1..20: mol_type = other RNA
tgtgctagacatgaggtcta

SEQ ID NO: 179 - RNA, 20 nt, synthetic construct
  modified_base 2: mod_base = OTHER; note = thymine
  modified_base 4: mod_base = OTHER; note = thymine
  modified_base 9: mod_base = OTHER; note = thymine
  modified_base 12: mod_base = OTHER; note = thymine
  misc_feature 1..20: note = TRAC sg11
  source 1..20: mol_type = other RNA
ctctcagctggtacacggca

SEQ ID NO: 180 - RNA, 20 nt, synthetic construct
  modified_base 12: mod_base = OTHER; note = thymine
  modified_base 18..19: mod_base = OTHER; note = thymine
  misc_feature 1..20: note = TRAC sg12
  source 1..20: mol_type = other RNA
acacggcagggtcagggttc

SEQ ID NO: 181 - RNA, 20 nt, synthetic construct
  modified_base 4: mod_base = OTHER; note = thymine
  modified_base 7: mod_base = OTHER; note = thymine
  modified_base 19: mod_base = OTHER; note = thymine
  misc_feature 1..20: note = TRAC sg13
  source 1..20: mol_type = other RNA
agctggtacacggcagggtc

SEQ ID NO: 182 - RNA, 20 nt, synthetic construct
  modified_base 6: mod_base = OTHER; note = thymine
  modified_base 12: mod_base = OTHER; note = thymine
  modified_base 16: mod_base = OTHER; note = thymine
  modified_base 20: mod_base = OTHER; note = thymine
  misc_feature 1..20: note = TRAC sg14
  source 1..20: mol_type = other RNA
gagaatcaaaatcggtgaat

SEQ ID NO: 183 - RNA, 20 nt, synthetic construct
  modified_base 7..8: mod_base = OTHER; note = thymine
  modified_base 10..11: mod_base = OTHER; note = thymine
  misc_feature 1..20: note = TRAC sg15
  source 1..20: mol_type = other RNA
gacaccttcttccccagccc

SEQ ID NO: 184 - RNA, 20 nt, synthetic construct
  modified_base 1: mod_base = OTHER; note = thymine
  modified_base 3: mod_base = OTHER; note = thymine
  modified_base 5: mod_base = OTHER; note = thymine
  modified_base 10: mod_base = OTHER; note = thymine
  modified_base 13: mod_base = OTHER; note = thymine
  misc_feature 1..20: note = TRAC sg16
  source 1..20: mol_type = other RNA
tctctcagctggtacacggc

SEQ ID NO: 185 - RNA, 20 nt, synthetic construct
  modified_base 3: mod_base = OTHER; note = thymine
  modified_base 6: mod_base = OTHER; note = thymine
  modified_base 18: mod_base = OTHER; note = thymine
  misc_feature 1..20: note = TRAC sg17
  source 1..20: mol_type = other RNA
gctggtacacggcagggtca

SEQ ID NO: 186 - RNA, 20 nt, synthetic construct
  modified_base 5: mod_base = OTHER; note = thymine
  modified_base 10..12: mod_base = OTHER; note = thymine
  modified_base 14..15: mod_base = OTHER; note = thymine
  modified_base 18: mod_base = OTHER; note = thymine
  misc_feature 1..20: note = TRAC sg18
  source 1..20: mol_type = other RNA
aaagtcagatttgttgctcc

SEQ ID NO: 187 - RNA, 20 nt, synthetic construct
  modified_base 2: mod_base = OTHER; note = thymine
  modified_base 14: mod_base = OTHER; note = thymine
  modified_base 16: mod_base = OTHER; note = thymine
  modified_base 18..19: mod_base = OTHER; note = thymine
  misc_feature 1..20: note = TRAC sg19
  source 1..20: mol_type = other RNA
ctggggaagaaggtgtcttc

SEQ ID NO: 188 - RNA, 20 nt, synthetic construct
  modified_base 1: mod_base = OTHER; note = thymine
  modified_base 5..7: mod_base = OTHER; note = thymine
  modified_base 12: mod_base = OTHER; note = thymine
  modified_base 14: mod_base = OTHER; note = thymine
  modified_base 16: mod_base = OTHER; note = thymine
  misc_feature 1..20: note = TRAC sg20
  source 1..20: mol_type = other RNA
tggatttagagtctctcagc

SEQ ID NO: 189 - RNA, 20 nt, synthetic construct
  modified_base 11: mod_base = OTHER; note = thymine
  modified_base 14: mod_base = OTHER; note = thymine
  modified_base 16: mod_base = OTHER; note = thymine
  misc_feature 1..20: note = TRAC sg21
  source 1..20: mol_type = other RNA
agagcaacagtgctgtggcc

SEQ ID NO: 190 - RNA, 20 nt, synthetic construct
  modified_base 2..3: mod_base = OTHER; note = thymine
  modified_base 16: mod_base = OTHER; note = thymine
  modified_base 19: mod_base = OTHER; note = thymine
  misc_feature 1..20: note = TRAC sg22
  source 1..20: mol_type = other RNA
cttcaagagcaacagtgctg

SEQ ID NO: 191 - RNA, 20 nt, synthetic construct
  modified_base 2..4: mod_base = OTHER; note = thymine
  modified_base 6..8: mod_base = OTHER; note = thymine
  modified_base 14: mod_base = OTHER; note = thymine
  modified_base 20: mod_base = OTHER; note = thymine
  misc_feature 1..20: note = TRAC sg23
  source 1..20: mol_type = other RNA
atttgtttgagaatcaaaat

SEQ ID NO: 192 - RNA, 20 nt, synthetic construct
  modified_base 4: mod_base = OTHER; note = thymine
  modified_base 7: mod_base = OTHER; note = thymine
  modified_base 10: mod_base = OTHER; note = thymine
  modified_base 13: mod_base = OTHER; note = thymine
  modified_base 16: mod_base = OTHER; note = thymine
  modified_base 18: mod_base = OTHER; note = thymine
  misc_feature 1..20: note = HLA-A02 sg10
  source 1..20: mol_type = other RNA
ccctcgtcctgctactctcg

SEQ ID NO: 193 - RNA, 20 nt, synthetic construct
  modified_base 3: mod_base = OTHER; note = thymine
  modified_base 6: mod_base = OTHER; note = thymine
  modified_base 9: mod_base = OTHER; note = thymine
  modified_base 12: mod_base = OTHER; note = thymine
  misc_feature 1..20: note = HLA-A02 sg2
  source 1..20: mol_type = other RNA
cgtactggtggtacccgcgg

SEQ ID NO: 194 - RNA, 20 nt, synthetic construct
  modified_base 2: mod_base = OTHER; note = thymine
  modified_base 8: mod_base = OTHER; note = thymine
  modified_base 19: mod_base = OTHER; note = thymine
  misc_feature 1..20: note = HLA-A02 sg5
  source 1..20: mol_type = other RNA
ctgaccatgaagccaccctg

SEQ ID NO: 195 - RNA, 20 nt, synthetic construct
  modified_base 5: mod_base = OTHER; note = thymine
  modified_base 13: mod_base = OTHER; note = thymine
  modified_base 19: mod_base = OTHER; note = thymine
  misc_feature 1..20: note = HLA-A02 sg14
  source 1..20: mol_type = other RNA
agactcaccgagtggacctg

SEQ ID NO: 196 - RNA, 20 nt, synthetic construct
  modified_base 7: mod_base = OTHER; note = thymine
  modified_base 10: mod_base = OTHER; note = thymine
  modified_base 13: mod_base = OTHER; note = thymine
  modified_base 15: mod_base = OTHER; note = thymine
  modified_base 17: mod_base = OTHER; note = thymine
  misc_feature 1..20: note = HLA-A02 sg21
  source 1..20: mol_type = other RNA
ggaccctcctgctctatcca

SEQ ID NO: 197 - RNA, 20 nt, synthetic construct
  modified_base 3: mod_base = OTHER; note = thymine
  modified_base 5: mod_base = OTHER; note = thymine
  modified_base 8: mod_base = OTHER; note = thymine
  modified_base 11..12: mod_base = OTHER; note = thymine
  modified_base 17: mod_base = OTHER; note = thymine
  modified_base 20: mod_base = OTHER; note = thymine
  misc_feature 1..20: note = HLA-A02 sg23
  source 1..20: mol_type = other RNA
gatgtaatccttgccgtcgt

SEQ ID NO: 198 - RNA, 20 nt, synthetic construct
  modified_base 3: mod_base = OTHER; note = thymine
  modified_base 8: mod_base = OTHER; note = thymine
  modified_base 10..11: mod_base = OTHER; note = thymine
  misc_feature 1..20: note = HLA-A02 sg26
  source 1..20: mol_type = other RNA
cctgcgctcttggaccgcgg

SEQ ID NO: 199 - RNA, 20 nt, synthetic construct
  modified_base 3: mod_base = OTHER; note = thymine
  modified_base 6: mod_base = OTHER; note = thymine
  modified_base 9: mod_base = OTHER; note = thymine
  modified_base 12: mod_base = OTHER; note = thymine
  modified_base 15: mod_base = OTHER; note = thymine
  modified_base 17: mod_base = OTHER; note = thymine
  misc_feature 1..20: note = HLA-A02 sg29
  source 1..20: mol_type = other RNA
cctcgtcctgctactctcgg

SEQ ID NO: 200 - RNA, 20 nt, synthetic construct
  modified_base 6: mod_base = OTHER; note = thymine
  modified_base 9: mod_base = OTHER; note = thymine
  modified_base 12: mod_base = OTHER; note = thymine
  modified_base 15: mod_base = OTHER; note = thymine
  modified_base 18: mod_base = OTHER; note = thymine
  modified_base 20: mod_base = OTHER; note = thymine
  misc_feature 1..20: note = HLA-A02 sg30
  source 1..20: mol_type = other RNA
aaccctcgtcctgctactct

SEQ ID NO: 201 - RNA, 20 nt, synthetic construct
  modified_base 6..7: mod_base = OTHER; note = thymine
  modified_base 18: mod_base = OTHER; note = thymine
  misc_feature 1..20: note = HLA-A02 sg31
  source 1..20: mol_type = other RNA
gagggttcggggcgccatga

SEQ ID NO: 202 - RNA, 20 nt, synthetic construct
  modified_base 3: mod_base = OTHER; note = thymine
  modified_base 6: mod_base = OTHER; note = thymine
  modified_base 9: mod_base = OTHER; note = thymine
  modified_base 11: mod_base = OTHER; note = thymine
  modified_base 19: mod_base = OTHER; note = thymine
  misc_feature 1..20: note = HLA-A02 sg32
  source 1..20: mol_type = other RNA
cctgctactctcgggggctc

SEQ ID NO: 203 - RNA, 20 nt, synthetic construct
  modified_base 2: mod_base = OTHER; note = thymine
  modified_base 5..6: mod_base = OTHER; note = thymine
  modified_base 8: mod_base = OTHER; note = thymine
  modified_base 11: mod_base = OTHER; note = thymine
  misc_feature 1..20: note = HLA-A02 sg33
  source 1..20: mol_type = other RNA
ctggttgtagtagccgcgca

SEQ ID NO: 204 - RNA, 20 nt, synthetic construct
  modified_base 1: mod_base = OTHER; note = thymine
  modified_base 9: mod_base = OTHER; note = thymine
  modified_base 14: mod_base = OTHER; note = thymine
  misc_feature 1..20: note = HLA-A02 sg34
  source 1..20: mol_type = other RNA
tagcccactgcgatgaagcg

SEQ ID NO: 205 - RNA, 20 nt, synthetic construct
  modified_base 2: mod_base = OTHER; note = thymine
  modified_base 8: mod_base = OTHER; note = thymine
  modified_base 17: mod_base = OTHER; note = thymine
  misc_feature 1..20: note = HLA-A02 sg35
  source 1..20: mol_type = other RNA
gtggacctggggaccctgcg

SEQ ID NO: 206 - RNA, 20 nt, synthetic construct
  modified_base 1: mod_base = OTHER; note = thymine
  modified_base 15..16: mod_base = OTHER; note = thymine
  modified_base 19: mod_base = OTHER; note = thymine
  misc_feature 1..20: note = HLA-A02 sg36
  source 1..20: mol_type = other RNA
tggacgacacgcagttcgtg

SEQ ID NO: 207 - RNA, 20 nt, synthetic construct
  modified_base 7: mod_base = OTHER; note = thymine
  modified_base 15: mod_base = OTHER; note = thymine
  misc_feature 1..20: note = HLA-A02 sg37
  source 1..20: mol_type = other RNA
acagactcaccgagtggacc

SEQ ID NO: 208 - RNA, 20 nt, synthetic construct
  modified_base 10: mod_base = OTHER; note = thymine
  modified_base 17: mod_base = OTHER; note = thymine
  modified_base 19..20: mod_base = OTHER; note = thymine
  misc_feature 1..20: note = HLA-A02 sg38
  source 1..20: mol_type = other RNA
gcaggagggtccggagtatt

SEQ ID NO: 209 - RNA, 20 nt, synthetic construct
  modified_base 3: mod_base = OTHER; note = thymine
  modified_base 5..6: mod_base = OTHER; note = thymine
  misc_feature 1..20: note = HLA-A02 sg39
  source 1..20: mol_type = other RNA
agtattgggacggggagaca

SEQ ID NO: 210 - RNA, 20 nt, synthetic construct
  modified_base 2: mod_base = OTHER; note = thymine
  misc_feature 1..20: note = HLA-A02 sg40
  source 1..20: mol_type = other RNA
ctcagaccaccaagcacaag

SEQ ID NO: 211 - RNA, 20 nt, synthetic construct
  modified_base 10: mod_base = OTHER; note = thymine
  misc_feature 1..20: note = HLA-A02 sg41
  source 1..20: mol_type = other RNA
ccgccgcggtccaagagcgc

SEQ ID NO: 212 - RNA, 20 nt, synthetic construct
  modified_base 2: mod_base = OTHER; note = thymine
  modified_base 4..5: mod_base = OTHER; note = thymine
  misc_feature 1..20: note = HLA-A02 sg42
  source 1..20: mol_type = other RNA
ctcttggaccgcggcggaca

SEQ ID NO: 213 - RNA, 20 nt, synthetic construct
  modified_base 4..5: mod_base = OTHER; note = thymine
  modified_base 9: mod_base = OTHER; note = thymine
  modified_base 15: mod_base = OTHER; note = thymine
  misc_feature 1..20: note = HLA-A02 sg43
  source 1..20: mol_type = other RNA
ggattacatcgccctgaaag

SEQ ID NO: 214 - RNA, 20 nt, synthetic construct
  modified_base 11: mod_base = OTHER; note = thymine
  misc_feature 1..20: note = HLA-A11 sg8-3
  source 1..20: mol_type = other RNA
cccccgagagtagcaggagg

SEQ ID NO: 215 - RNA, 20 nt, synthetic construct
  modified_base 3: mod_base = OTHER; note = thymine
  modified_base 17..18: mod_base = OTHER; note = thymine
  misc_feature 1..20: note = HLA-A11 sg9-3
  source 1..20: mol_type = other RNA
agtagcaggaggagggttcg

SEQ ID NO: 216 - RNA, 20 nt, synthetic construct
  modified_base 4: mod_base = OTHER; note = thymine
  modified_base 7: mod_base = OTHER; note = thymine
  modified_base 10: mod_base = OTHER; note = thymine
  modified_base 13: mod_base = OTHER; note = thymine
  modified_base 16: mod_base = OTHER; note = thymine
  modified_base 18: mod_base = OTHER; note = thymine
  misc_feature 1..20: note = HLA-A11 sg10-3
  source 1..20: mol_type = other RNA
ccctcctcctgctactctcg

SEQ ID NO: 217 - RNA, 20 nt, synthetic construct
  modified_base 10: mod_base = OTHER; note = thymine
  misc_feature 1..20: note = HLA-A11 sg11-3
  source 1..20: mol_type = other RNA
ccccgagagtagcaggagga

SEQ ID NO: 218 - RNA, 20 nt, synthetic construct
  modified_base 5: mod_base = OTHER; note = thymine
  modified_base 13: mod_base = OTHER; note = thymine
  modified_base 19: mod_base = OTHER; note = thymine
  misc_feature 1..20: note = HLA-A11 sg14-3
  source 1..20: mol_type = other RNA
agactgaccgagtggacctg

SEQ ID NO: 219 - RNA, 20 nt, synthetic construct
  modified_base 11: mod_base = OTHER; note = thymine
  modified_base 13..14: mod_base = OTHER; note = thymine
  misc_feature 1..20: note = HLA-A11 sg16-3
  source 1..20: mol_type = other RNA
ggggccggagtattgggacc

SEQ ID NO: 220 - RNA, 20 nt, synthetic construct
  modified_base 5: mod_base = OTHER; note = thymine
  modified_base 9: mod_base = OTHER; note = thymine
  modified_base 13: mod_base = OTHER; note = thymine
  modified_base 15: mod_base = OTHER; note = thymine
  modified_base 17: mod_base = OTHER; note = thymine
  misc_feature 1..20: note = HLA-A11 sg20-3
  source 1..20: mol_type = other RNA
ccactcggtcagtctgtgac

SEQ ID NO: 221 - RNA, 20 nt, synthetic construct
  modified_base 1: mod_base = OTHER; note = thymine
  modified_base 5: mod_base = OTHER; note = thymine
  misc_feature 1..20: note = HLA-A11 sg21-3
  source 1..20: mol_type = other RNA
tggatagagcaggaggggcc

SEQ ID NO: 222 - RNA, 20 nt, synthetic construct
  modified_base 1: mod_base = OTHER; note = thymine
  modified_base 6: mod_base = OTHER; note = thymine
  modified_base 9: mod_base = OTHER; note = thymine
  modified_base 15: mod_base = OTHER; note = thymine
  modified_base 18: mod_base = OTHER; note = thymine
  misc_feature 1..20: note = HLA-A11 sg28-3
  source 1..20: mol_type = other RNA
tgccgtcgtaggcgtcctgc

SEQ ID NO: 223 - RNA, 20 nt, synthetic construct
  modified_base 3: mod_base = OTHER; note = thymine
  modified_base 6: mod_base = OTHER; note = thymine
  modified_base 12: mod_base = OTHER; note = thymine
  misc_feature 1..20: note = HLA-A11 Rsg2
  source 1..20: mol_type = other RNA
cgtcctgccggtacccgcgg

SEQ ID NO: 224 - RNA, 20 nt, synthetic construct
  modified_base 7: mod_base = OTHER; note = thymine
  modified_base 10: mod_base = OTHER; note = thymine
  modified_base 13: mod_base = OTHER; note = thymine
  modified_base 15: mod_base = OTHER; note = thymine
  modified_base 17: mod_base = OTHER; note = thymine
  misc_feature 1..20: note = HLA-A11 sg21
  source 1..20: mol_type = other RNA
ggcccctcctgctctatcca

SEQ ID NO: 225 - RNA, 20 nt, synthetic construct
  modified_base 3: mod_base = OTHER; note = thymine
  modified_base 9: mod_base = OTHER; note = thymine
  modified_base 20: mod_base = OTHER; note = thymine
  misc_feature 1..20: note = HLA-A24 sg12-2
  source 1..20: mol_type = other RNA
cctggccctgacccagacct

SEQ ID NO: 226 - RNA, 20 nt, synthetic construct
  modified_base 4: mod_base = OTHER; note = thymine
  modified_base 10: mod_base = OTHER; note = thymine
  misc_feature 1..20: note = HLA-A24 sg13-2
  source 1..20: mol_type = other RNA
ccctggccctgacccagacc

SEQ ID NO: 227 - RNA, 20 nt, synthetic construct
  modified_base 5: mod_base = OTHER; note = thymine
  modified_base 19: mod_base = OTHER; note = thymine
  misc_feature 1..20: note = HLA-A24 sg14-2
  source 1..20: mol_type = other RNA
agactgaccgagagaacctg

SEQ ID NO: 228 - RNA, 20 nt, synthetic construct
  modified_base 11: mod_base = OTHER; note = thymine
  modified_base 13..14: mod_base = OTHER; note = thymine
  misc_feature 1..20: note = HLA-A24 sg16-2
  source 1..20: mol_type = other RNA
ggggccggagtattgggacg

SEQ ID NO: 229 - RNA, 20 nt, synthetic construct
  modified_base 1: mod_base = OTHER; note = thymine
  modified_base 3: mod_base = OTHER; note = thymine
  modified_base 5: mod_base = OTHER; note = thymine
  modified_base 9: mod_base = OTHER; note = thymine
  modified_base 13: mod_base = OTHER; note = thymine
  modified_base 15: mod_base = OTHER; note = thymine
  modified_base 17: mod_base = OTHER; note = thymine
  misc_feature 1..20: note = HLA-A24 sg20-2
  source 1..20: mol_type = other RNA
tctctcggtcagtctgtgag

SEQ ID NO: 230 - RNA, 20 nt, synthetic construct
  modified_base 7: mod_base = OTHER; note = thymine
  modified_base 10: mod_base = OTHER; note = thymine
  modified_base 13: mod_base = OTHER; note = thymine
  modified_base 15: mod_base = OTHER; note = thymine
  modified_base 17: mod_base = OTHER; note = thymine
  misc_feature 1..20: note = HLA-A24 sg21-2
  source 1..20: mol_type = other RNA
ggcccctcctgctctatcca

SEQ ID NO: 231 - RNA, 20 nt, synthetic construct
  modified_base 6: mod_base = OTHER; note = thymine
  modified_base 9: mod_base = OTHER; note = thymine
  modified_base 12: mod_base = OTHER; note = thymine
  modified_base 15: mod_base = OTHER; note = thymine
  misc_feature 1..20: note = HLA-A24 sg22-2
  source 1..20: mol_type = other RNA
aggcgtactggtggtacccg

SEQ ID NO: 232 - RNA, 20 nt, synthetic construct
  modified_base 2: mod_base = OTHER; note = thymine
  modified_base 12: mod_base = OTHER; note = thymine
  modified_base 14: mod_base = OTHER; note = thymine
  misc_feature 1..20: note = HLA-A24 sg25-2
  source 1..20: mol_type = other RNA
ctgagccgccatgtccgccg

SEQ ID NO: 233 - RNA, 21 nt, synthetic construct
  modified_base 10..11: mod_base = OTHER; note = thymine
  modified_base 19: mod_base = OTHER; note = thymine
  misc_feature 1..21: note = HLA-A-homo-551
  source 1..21: mol_type = other RNA
gcggagcagttgagagcctac

SEQ ID NO: 234 - RNA, 21 nt, synthetic construct
  modified_base 3: mod_base = OTHER; note = thymine
  modified_base 8: mod_base = OTHER; note = thymine
  misc_feature 1..21: note = HLA-A-homo-NEG
  source 1..21: mol_type = other RNA
gctcagatcaccaagcgcaag

SEQ ID NO: 235 - RNA, 21 nt, synthetic construct
  modified_base 6: mod_base = OTHER; note = thymine
  modified_base 14..16: mod_base = OTHER; note = thymine
  modified_base 19: mod_base = OTHER; note = thymine
  modified_base 21: mod_base = OTHER; note = thymine
  misc_feature 1..21: note = TRAC-homo-375
  source 1..21: mol_type = other RNA
gaaagtggccgggtttaatct

SEQ ID NO: 236 - RNA, 21 nt, synthetic construct
  modified_base 9: mod_base = OTHER; note = thymine
  modified_base 17: mod_base = OTHER; note = thymine
  misc_feature 1..21: note = TRAC-homo-NEG
  source 1..21: mol_type = other RNA
gaaacagatacgaacctaaac

SEQ ID NO: 237 - RNA, 20 nt, synthetic construct
  modified_base 3: mod_base = OTHER; note = thymine
  modified_base 5: mod_base = OTHER; note = thymine
  misc_feature 1..20: note = HLA-B40 Sg6
  source 1..20: mol_type = other RNA
catgtcccggcccggccgcg

SEQ ID NO: 238 - RNA, 20 nt, synthetic construct
  modified_base 14: mod_base = OTHER; note = thymine
  modified_base 17: mod_base = OTHER; note = thymine
  misc_feature 1..20: note = HLA-B40 Sg19
  source 1..20: mol_type = other RNA
ccggacgggcgcctcctccg

SEQ ID NO: 239 - RNA, 20 nt, synthetic construct
  modified_base 2: mod_base = OTHER; note = thymine
  modified_base 8: mod_base = OTHER; note = thymine
  modified_base 17: mod_base = OTHER; note = thymine
  misc_feature 1..20: note = HLA-B46 Sg14
  source 1..20: mol_type = other RNA
gtgagcctgcggaacctgcg

SEQ ID NO: 240 - DNA, 2235 bp, synthetic construct
  misc_feature 1..2235: note = The nucleic acids encoding the 1st polypeptide
  source 1..2235: mol_type = other DNA
atggccttaccagtgaccgccttgctcctgccgctggccttgctgctccacgccgccaggccggctgtccagcttgtggagtctggggggggcctcgtccagacaggcggttctctccgcctctcctgtgctgattctggcagaatcttttcaaactacgcaatgggctggttcaggcaggcaccaggcaaggagcgggagttcgtggctgctatcattggatctactggcaccgttaactacgcagacagcatgaaaggcagatttaccatctcaagagataacgccaaaaatactgtagtcctccagatgaactctctgaagcctgaggataccgctatatattattgtgcggcgtcattcaggtacagcggcatctatggccgcgaagcggattttgttagttggggacaagggacccaagtgacagtgtcttcaggaggcggaggttctggcggcggaggaagtggtggcggaggctctcaggctcaactggtggagtcgggaggtggcttggtgcagacaggagggagcctgcgactctcctgtgcggcttccggaaggattttctctaattattctgtcggatggttccggcaggccccaggcaaagagcgtgaattcgttgcggcgataatctggtcgaccggaacaacgaatctggccgatcccatgaaggggagattcaccattagtagagacaacgcaaaaaacacagtagtcctgcagatgaacagcctcaaacccgaggatacagctatctattactgcgcagcttcctttaaatattctggcatatatggcagagaagcagattttgggagttgggggcagggcacccaggtgacagtcagttctttcgtccccgtgttcctgcctgccaagccaacaactacccctgctccacgaccacctactccagcacctaccatcgcaagtcagcccctgtcactgcgacctgaggcttgccggccagcagctggaggagcagtgcacacccgaggcctggacttcgcatgcgatatctacatttgggcaccactggctggaacctgtggggtcctgctgctgagcctggtcatcaccctgtattgtaaccacagaaataaaagggggcgcaagaaactgctgtacatcttcaagcagccttttatgcgcccagtgcagacaactcaggaggaagacggatgctcttgtcggttcccagaggaggaggaaggaggctgcgagctgagagtgaagttcagccggagcgccgatgcaccagcatatcagcagggacagaatcagctgtacaacgagctgaatctgggcaggcgcgaggaatatgacgtgctggataagcgacgaggacgggaccccgaaatgggaggaaaacccagaaggaagaaccctcaggaggggctgtataatgaactgcagaaagacaagatggctgaggcatacagcgaaattggaatgaaaggagagcgccgacgggggaagggacacgatgggctgtaccagggactgtcaaccgccactaaagatacctacgacgcactgcacatgcaggctctgcccccaagagagggcagaggcagcctgctgacatgtggcgacgtggaagagaaccctggccccatggccttaccagtgaccgccttgctcctgccgctggccttgctgctccacgccgccaggccgaactgggtgaatgtaataagtgatttgaaaaaaattgaagatcttattcaatctatgcatattgatgctactttatatacggaaagtgatgttcaccccagttgcaaagtaacagcaatgaagtgctttctcttggagttacaagttatttcacttgagtccggagatgcaagtattcatgatacagtagaaaatctgatcatcctagcaaacaacagtttgtcttctaatgggaatgtaacagaatctggatgcaaagaatgtgaggaactggaggaaaaaaatattaaagaatttttgcagagttttgtacatattgtccaaatgttcatcaacacttctaccacgacgccagcgccgcgaccaccaacaccggcgcccaccatcgcgtcgcagcccctgtccctgcgcccagaggcgtgccggccagcggcggggggcgcagtgcacacgagggggctggacttcgcctgtgatatctacatctgggcgcccttggccgggacttgtggggtccttctcctgtcactggttatcaccctttactgc

SEQ ID NO: 241 - protein, 745 aa, synthetic construct
  REGION 1..745: note = The 1st polypeptide
MALPVTALLLPLALLLHAARPAVQLVESGGGLVQTGGSLRLSCADSGRIFSNYAMGWFRQAPGKEREFVAAIIGSTGTVNYADSMKGRFTISRDNAKNTVVLQMNSLKPEDTAIYYCAASFRYSGIYGREADFVSWGQGTQVTVSSGGGGSGGGGSGGGGSQAQLVESGGGLVQTGGSLRLSCAASGRIFSNYSVGWFRQAPGKEREFVAAIIWSTGTTNLADPMKGRFTISRDNAKNTVVLQMNSLKPEDTAIYYCAASFKYSGIYGREADFGSWGQGTQVTVSSFVPVFLPAKPTTTPAPRPPTPAPTIASQPLSLRPEACRPAAGGAVHTRGLDFACDIYIWAPLAGTCGVLLLSLVITLYCNHRNKRGRKKLLYIFKQPFMRPVQTTQEEDGCSCRFPEEEEGGCELRVKFSRSADAPAYQQGQNQLYNELNLGRREEYDVLDKRRGRDPEMGGKPRRKNPQEGLYNELQKDKMAEAYSEIGMKGERRRGKGHDGLYQGLSTATKDTYDALHMQALPPREGRGSLLTCGDVEENPGPMALPVTALLLPLALLLHAARPNWVNVISDLKKIEDLIQSMHIDATLYTESDVHPSCKVTAMKCFLLELQVISLESGDASIHDTVENLIILANNSLSSNGNVTESGCKECEELEEKNIKEFLQSFVHIVQMFINTSTTTPAPRPPTPAPTIASQPLSLRPEACRPAAGGAVHTRGLDFACDIYIWAPLAGTCGVLLLSLVITLYC

SEQ ID NO: 242 - DNA, 2808 bp, synthetic construct
  misc_feature 1..2808: note = The nucleic acids encoding the 2nd polypeptide
  source 1..2808: mol_type = other DNA
atggccttaccagtgaccgccttgctcctgccgctggccttgctgctccacgccgccaggccggctgtccagcttgtggagtctggggggggcctcgtccagacaggcggttctctccgcctctcctgtgctgattctggcagaatcttttcaaactacgcaatgggctggttcaggcaggcaccaggcaaggagcgggagttcgtggctgctatcattggatctactggcaccgttaactacgcagacagcatgaaaggcagatttaccatctcaagagataacgccaaaaatactgtagtcctccagatgaactctctgaagcctgaggataccgctatatattattgtgcggcgtcattcaggtacagcggcatctatggccgcgaagcggattttgttagttggggacaagggacccaagtgacagtgtcttcaggaggcggaggttctggcggcggaggaagtggtggcggaggctctcaggctcaactggtggagtcgggaggtggcttggtgcagacaggagggagcctgcgactctcctgtgcggcttccggaaggattttctctaattattctgtcggatggttccggcaggccccaggcaaagagcgtgaattcgttgcggcgataatctggtcgaccggaacaacgaatctggccgatcccatgaaggggagattcaccattagtagagacaacgcaaaaaacacagtagtcctgcagatgaacagcctcaaacccgaggatacagctatctattactgcgcagcttcctttaaatattctggcatatatggcagagaagcagattttgggagttgggggcagggcacccaggtgacagtcagttctttcgtccccgtgttcctgcctgccaagccaacaactacccctgctccacgaccacctactccagcacctaccatcgcaagtcagcccctgtcactgcgacctgaggcttgccggccagcagctggaggagcagtgcacacccgaggcctggacttcgcatgcgatatctacatttgggcaccactggctggaacctgtggggtcctgctgctgagcctggtcatcaccctgtattgtaaccacagaaataaaagggggcgcaagaaactgctgtacatcttcaagcagccttttatgcgcccagtgcagacaactcaggaggaagacggatgctcttgtcggttcccagaggaggaggaaggaggctgcgagctgagagtgaagttcagccggagcgccgatgcaccagcatatcagcagggacagaatcagctgtacaacgagctgaatctgggcaggcgcgaggaatatgacgtgctggataagcgacgaggacgggaccccgaaatgggaggaaaacccagaaggaagaaccctcaggaggggctgtataatgaactgcagaaagacaagatggctgaggcatacagcgaaattggaatgaaaggagagcgccgacgggggaagggacacgatgggctgtaccagggactgtcaaccgccactaaagatacctacgacgcactgcacatgcaggctctgcccccaagagagggcagaggcagcctgctgacatgtggcgacgtggaagagaaccctggccccatggactggacgtggatcttgttcctggttgcagcagcaactcgtgtgcacagtaattgggtgaacgtcatcagcgatctgaaaaaaatagaagatctgattcagtccatgcatattgacgctacactctacacggagtccgacgtgcatccgtcctgcaaggtgaccgccatgaaatgtttcctgttggagctgcaggtcatcagcctcgagagcggagatgcttcaatacacgacaccgtcgagaatttgattattttggcaaataattccttgtcgtctaacggcaatgtcactgaaagcggttgcaaagagtgtgaagaattggaagaaaagaatatcaaggagtttctccagtcttttgttcatattgttcagatgttcatcaacacatcgagtggcggcggcagcggtggggggggttctggcggcggcggctccggaggtggtgggtccggtggaggtagtctgcagatcacttgtccacctcctatgtcagtggagcatgcggacatttgggtgaagagctacagtttatactcccgcgaaaggtacatctgcaatagcggattcaaacgcaaagcaggcacttcatcactcactgagtgtgtgttgaataaggcaaccaacgtggctcattggacaactccttccctgaagtgcattcgagaccccgccctcgtccatcagcgcccagccccaccttctacagtcaccaccgccggcgtgacacctcagcccgaaagccttagcccttccgggaaagaaccagctgcttctagcccctcatcaaacaataccgccgctactacagccgccattgtcccaggaagccagctgatgccgtccaagagccccagtactgggaccactgaaatctcctcccatgaaagctcccacgggactccgagtcagaccaccgcaaaaaattgggagctgactgctagcgcatcacaccagccccccggtgtgtatccacagggtcactctgatactacggttgctataagcacgagtactgtattactgtgcggtctgtccgccgtctctctgctggcctgctatctgaagtcccggcaaacacccccccttgcgtcagtggaaatggaagccatggaggcattgccggtgacgtggggaacttcatctagggacgaggacctggaaaactgtagccaccacctc

SEQ ID NO: 243 - protein, 936 aa, synthetic construct
  REGION 1..936: note = The 2nd polypeptide
MALPVTALLLPLALLLHAARPAVQLVESGGGLVQTGGSLRLSCADSGRIFSNYAMGWFRQAPGKEREFVAAIIGSTGTVNYADSMKGRFTISRDNAKNTVVLQMNSLKPEDTAIYYCAASFRYSGIYGREADFVSWGQGTQVTVSSGGGGSGGGGSGGGGSQAQLVESGGGLVQTGGSLRLSCAASGRIFSNYSVGWFRQAPGKEREFVAAIIWSTGTTNLADPMKGRFTISRDNAKNTVVLQMNSLKPEDTAIYYCAASFKYSGIYGREADFGSWGQGTQVTVSSFVPVFLPAKPTTTPAPRPPTPAPTIASQPLSLRPEACRPAAGGAVHTRGLDFACDIYIWAPLAGTCGVLLLSLVITLYCNHRNKRGRKKLLYIFKQPFMRPVQTTQEEDGCSCRFPEEEEGGCELRVKFSRSADAPAYQQGQNQLYNELNLGRREEYDVLDKRRGRDPEMGGKPRRKNPQEGLYNELQKDKMAEAYSEIGMKGERRRGKGHDGLYQGLSTATKDTYDALHMQALPPREGRGSLLTCGDVEENPGPMDWTWILFLVAAATRVHSNWVNVISDLKKIEDLIQSMHIDATLYTESDVHPSCKVTAMKCFLLELQVISLESGDASIHDTVENLIILANNSLSSNGNVTESGCKECEELEEKNIKEFLQSFVHIVQMFINTSSGGGSGGGGSGGGGSGGGGSGGGSLQITCPPPMSVEHADIWVKSYSLYSRERYICNSGFKRKAGTSSLTECVLNKATNVAHWTTPSLKCIRDPALVHQRPAPPSTVTTAGVTPQPESLSPSGKEPAASSPSSNNTAATTAAIVPGSQLMPSKSPSTGTTEISSHESSHGTPSQTTAKNWELTASASHQPPGVYPQGHSDTTVAISTSTVLLCGLSAVSLLACYLKSRQTPPLASVEMEAMEALPVTWGTSSRDEDLENCSHHL

SEQ ID NO: 244 - protein, 265 aa, synthetic construct
  REGION 1..265: note = Hbrca84d-2
MALPVTALLLPLALLLHAARPEVQLVESGGGLVQPGGSLRLSCAASGFTFSSFGMHWVRQAPGKGLEWVAYISSDSSAIYYADTVKGRFTISRDNAKNSLYLQMNSLRDEDTAVYYCGRGRENIYYGSRLDYWGQGTTVTVSSGGGGSGGGGSGGGGSDIQLTQSPSFLSASVGDRVTITCKASQNVDTNVAWYQQKPGKAPKALIYSASYRYSGVPSRFSGSGSGTDFTLTISSLQPEDFATYYCQQYNNYPFTFGQGTKLEIK